European Patent Specification EP 4 277 648 B1, published July 29, 2026. Title: TREATMENT OF BRAIN DAMAGE. Applicant: IPSEN BIOPHARM LIMITED. The sequence listing filed with the application follows.

SEQUENCE LISTING (76 sequences)

SEQ ID NO: 1 - DNA, 3888 bp, Artificial Sequence
  Nucleotide Sequence of rBoNT/A(0)
atgccattcgtcaacaagcaattcaactacaaagacccagtcaacggcgtcgacatcgcatacatcaagattccgaacgccggtcaaatgcagccggttaaggcttttaagatccacaacaagatttgggttatcccggagcgtgacaccttcacgaacccggaagaaggcgatctgaacccgccaccggaagcgaagcaagtccctgtcagctactacgattcgacgtacctgagcacggataacgaaaaagataactacctgaaaggtgtgaccaagctgttcgaacgtatctacagcacggatctgggtcgcatgctgctgactagcattgttcgcggtatcccgttctggggtggtagcacgattgacaccgaactgaaggttatcgacactaactgcattaacgttattcaaccggatggtagctatcgtagcgaagagctgaatctggtcatcattggcccgagcgcagacattatccaattcgagtgcaagagctttggtcacgaggttctgaatctgacccgcaatggctatggtagcacccagtacattcgtttttcgccggattttaccttcggctttgaagagagcctggaggttgataccaatccgttgctgggtgcgggcaaattcgctaccgatccggctgtcacgctggcccatcaactgatctacgcaggccaccgcctgtacggcattgccatcaacccaaaccgtgtgttcaaggttaatacgaatgcatactacgagatgagcggcctggaagtcagcttcgaagaactgcgcaccttcggtggccatgacgctaaattcattgacagcttgcaagagaatgagttccgtctgtactactataacaaattcaaagacattgcaagcacgttgaacaaggccaaaagcatcgttggtactaccgcgtcgttgcagtatatgaagaatgtgtttaaagagaagtacctgctgtccgaggatacctccggcaagtttagcgttgataagctgaagtttgacaaactgtacaagatgctgaccgagatttacaccgaggacaactttgtgaaattcttcaaagtgttgaatcgtaaaacctatctgaattttgacaaagcggttttcaagattaacatcgtgccgaaggtgaactacaccatctatgacggttttaacctgcgtaacaccaacctggcggcgaactttaacggtcagaatacggaaatcaacaacatgaatttcacgaagttgaagaacttcacgggtctgttcgagttctataagctgctgtgcgtgcgcggtatcatcaccagcaaaaccaaaagcctggacaaaggctacaacaaggcgctgaatgacctgtgcattaaggtaaacaattgggatctgttcttttcgccatccgaagataattttaccaacgacctgaacaagggtgaagaaatcaccagcgatacgaatattgaagcagcggaagagaatatcagcctggatctgatccagcagtactatctgacctttaacttcgacaatgaaccggagaacattagcattgagaatctgagcagcgacattatcggtcagctggaactgatgccgaatatcgaacgtttcccgaacggcaaaaagtacgagctggacaagtacactatgttccattacctgcgtgcacaggagtttgaacacggtaaaagccgtatcgcgctgaccaacagcgttaacgaggccctgctgaacccgagccgtgtctataccttcttcagcagcgactatgttaagaaagtgaacaaagccactgaggccgcgatgttcctgggctgggtggaacagctggtatatgacttcacggacgagacgagcgaagtgagcactaccgacaaaattgctgatattaccatcattatcccgtatattggtccggcactgaacattggcaacatgctgtacaaagacgattttgtgggtgccctgatcttctccggtgccgtgattctgctggagttcattccggagattgcgatcccggtgttgggtaccttcgcgctggtgtcctacatcgcgaataaggttctgacggttcagaccatcgataacgcgctgtcgaaacgtaatgaaaaatgggacgaggtttacaaatacattgttacgaattggctggcgaaagtcaatacccagatcgacctgatccgtaagaaaatgaaagaggcgctggagaatcaggcggaggccaccaaagcaattatcaactaccaatacaaccagtacacggaagaagagaagaataacattaacttcaatatcgatgatttgagcagcaagctgaatgaatctatcaacaaagcgatgatcaatatcaacaagtttttgaatcagtgtagcgtttcgtacctgatgaatagcatgattccgtatggcgtcaaacgtctggaggacttcgacgccagcctgaaagatgcgttgctgaaatacatttacgacaatcgtggtacgctgattggccaagttgaccgcttgaaagacaaagttaacaataccctgagcaccgacatcccatttcaactgagcaagtatgttgataatcaacgtctgttgagcactttcaccgagtatatcaaaaacatcatcaatactagcattctgaacctgcgttacgagagcaatcatctgattgatctgagccgttatgcaagcaagatcaacatcggtagcaaggtcaattttgacccgatcgataagaaccagatccagctgtttaatctggaatcgagcaaaattgaggttatcctgaaaaacgccattgtctacaactccatgtacgagaatttctccaccagcttctggattcgcatcccgaaatacttcaacagcattagcctgaacaacgagtatactatcatcaactgtatggagaacaacagcggttggaaggtgtctctgaactatggtgagatcatttggaccttgcaggacacccaagagatcaagcagcgcgtcgtgttcaagtactctcaaatgatcaacatttccgattacattaatcgttggatcttcgtgaccattacgaataaccgtctgaataacagcaagatttacatcaatggtcgcttgatcgatcagaaaccgattagcaacctgggtaatatccacgcaagcaacaacattatgttcaaattggacggttgccgcgatacccatcgttatatctggatcaagtatttcaacctgtttgataaagaactgaatgagaaggagatcaaagatttgtatgacaaccaatctaacagcggcattttgaaggacttctggggcgattatctgcaatacgataagccgtactatatgctgaacctgtatgatccgaacaaatatgtggatgtcaataatgtgggtattcgtggttacatgtatttgaagggtccgcgtggcagcgttatgacgaccaacatttacctgaactctagcctgtaccgtggtacgaaattcatcattaagaaatatgccagcggcaacaaagataacattgtgcgtaataacgatcgtgtctacatcaacgtggtcgtgaagaataaagagtaccgtctggcgaccaacgcttcgcaggcgggtgttgagaaaattctgagcgcgttggagatccctgatgtcggtaatctgagccaagtcgtggttatgaagagcaagaacgaccagggtatcactaacaagtgcaagatgaacctgcaagacaacaatggtaacgacatcggctttattggtttccaccagttcaacaatattgctaaactggtagcgagcaattggtacaatcgtcagattgagcgcagcagccgtactttgggctgtagctgggagtttatcccggtcgatgatggttggggcgaacgtccgctg

SEQ ID NO: 2 - protein, 1296 aa, Artificial Sequence
  Polypeptide Sequence of rBoNT/A(0)
MPFVNKQFNYKDPVNGVDIAYIKIPNAGQMQPVKAFKIHNKIWVIPERDTFTNPEEGDLNPPPEAKQVPVSYYDSTYLSTDNEKDNYLKGVTKLFERIYSTDLGRMLLTSIVRGIPFWGGSTIDTELKVIDTNCINVIQPDGSYRSEELNLVIIGPSADIIQFECKSFGHEVLNLTRNGYGSTQYIRFSPDFTFGFEESLEVDTNPLLGAGKFATDPAVTLAHQLIYAGHRLYGIAINPNRVFKVNTNAYYEMSGLEVSFEELRTFGGHDAKFIDSLQENEFRLYYYNKFKDIASTLNKAKSIVGTTASLQYMKNVFKEKYLLSEDTSGKFSVDKLKFDKLYKMLTEIYTEDNFVKFFKVLNRKTYLNFDKAVFKINIVPKVNYTIYDGFNLRNTNLAANFNGQNTEINNMNFTKLKNFTGLFEFYKLLCVRGIITSKTKSLDKGYNKALNDLCIKVNNWDLFFSPSEDNFTNDLNKGEEITSDTNIEAAEENISLDLIQQYYLTFNFDNEPENISIENLSSDIIGQLELMPNIERFPNGKKYELDKYTMFHYLRAQEFEHGKSRIALTNSVNEALLNPSRVYTFFSSDYVKKVNKATEAAMFLGWVEQLVYDFTDETSEVSTTDKIADITIIIPYIGPALNIGNMLYKDDFVGALIFSGAVILLEFIPEIAIPVLGTFALVSYIANKVLTVQTIDNALSKRNEKWDEVYKYIVTNWLAKVNTQIDLIRKKMKEALENQAEATKAIINYQYNQYTEEEKNNINFNIDDLSSKLNESINKAMININKFLNQCSVSYLMNSMIPYGVKRLEDFDASLKDALLKYIYDNRGTLIGQVDRLKDKVNNTLSTDIPFQLSKYVDNQRLLSTFTEYIKNIINTSILNLRYESNHLIDLSRYASKINIGSKVNFDPIDKNQIQLFNLESSKIEVILKNAIVYNSMYENFSTSFWIRIPKYFNSISLNNEYTIINCMENNSGWKVSLNYGEIIWTLQDTQEIKQRVVFKYSQMINISDYINRWIFVTITNNRLNNSKIYINGRLIDQKPISNLGNIHASNNIMFKLDGCRDTHRYIWIKYFNLFDKELNEKEIKDLYDNQSNSGILKDFWGDYLQYDKPYYMLNLYDPNKYVDVNNVGIRGYMYLKGPRGSVMTTNIYLNSSLYRGTKFIIKKYASGNKDNIVRNNDRVYINVVVKNKEYRLATNASQAGVEKILSALEIPDVGNLSQVVVMKSKNDQGITNKCKMNLQDNNGNDIGFIGFHQFNNIAKLVASNWYNRQIERSSRTLGCSWEFIPVDDGWGERPL

SEQ ID NO: 3 - DNA, 2634 bp, Artificial Sequence
  Nucleotide Sequence of rLHN/A
atggagttcgttaacaaacagttcaactataaagacccagttaacggtgttgacattgcttacatcaaaatcccgaacgctggccagatgcagccggtaaaggcattcaaaatccacaacaaaatctgggttatcccggaacgtgatacctttactaacccggaagaaggtgacctgaacccgccaccggaagcgaaacaggtgccggtatcttactatgactccacctacctgtctaccgataacgaaaaggacaactacctgaaaggtgttactaaactgttcgagcgtatttactccaccgacctgggccgtatgctgctgactagcatcgttcgcggtatcccgttctggggcggttctaccatcgataccgaactgaaagtaatcgacactaactgcatcaacgttattcagccggacggttcctatcgttccgaagaactgaacctggtgatcatcggcccgtctgctgatatcatccagttcgagtgtaagagctttggtcacgaagttctgaacctcacccgtaacggctacggttccactcagtacatccgtttctctccggacttcaccttcggttttgaagaatccctggaagtagacacgaacccactgctgggcgctggtaaattcgcaactgatcctgcggttaccctggctcacgaactgattcatgcaggccaccgcctgtacggtatcgccatcaatccgaaccgtgtcttcaaagttaacaccaacgcgtattacgagatgtccggtctggaagttagcttcgaagaactgcgtacttttggcggtcacgacgctaaattcatcgactctctgcaagaaaacgagttccgtctgtactactataacaagttcaaagatatcgcatccaccctgaacaaagcgaaatccatcgtgggtaccactgcttctctccagtacatgaagaacgtttttaaagaaaaatacctgctcagcgaagacacctccggcaaattctctgtagacaagttgaaattcgataaactttacaaaatgctgactgaaatttacaccgaagacaacttcgttaagttctttaaagttctgaaccgcaaaacctatctgaacttcgacaaggcagtattcaaaatcaacatcgtgccgaaagttaactacactatctacgatggtttcaacctgcgtaacaccaacctggctgctaattttaacggccagaacacggaaatcaacaacatgaacttcacaaaactgaaaaacttcactggtctgttcgagttttacaagctgctgtgcgtcgacggcatcattacctccaaaactaaatctgacgatgacgataaaaacaaagcgctgaacctgcagtgtatcaaggttaacaactgggatttattcttcagcccgagtgaagacaacttcaccaacgacctgaacaaaggtgaagaaatcacctcagatactaacatcgaagcagccgaagaaaacatctcgctggacctgatccagcagtactacctgacctttaatttcgacaacgagccggaaaacatttctatcgaaaacctgagctctgatatcatcggccagctggaactgatgccgaacatcgaacgtttcccaaacggtaaaaagtacgagctggacaaatataccatgttccactacctgcgcgcgcaggaatttgaacacggcaaatcccgtatcgcactgactaactccgttaacgaagctctgctcaacccgtcccgtgtatacaccttcttctctagcgactacgtgaaaaaggtcaacaaagcgactgaagctgcaatgttcttgggttgggttgaacagcttgtttatgattttaccgacgagacgtccgaagtatctactaccgacaaaattgcggatatcactatcatcatcccgtacatcggtccggctctgaacattggcaacatgctgtacaaagacgacttcgttggcgcactgatcttctccggtgcggtgatcctgctggagttcatcccggaaatcgccatcccggtactgggcacctttgctctggtttcttacattgcaaacaaggttctgactgtacaaaccatcgacaacgcgctgagcaaacgtaacgaaaaatgggatgaagtttacaaatatatcgtgaccaactggctggctaaggttaatactcagatcgacctcatccgcaaaaaaatgaaagaagcactggaaaaccaggcggaagctaccaaggcaatcattaactaccagtacaaccagtacaccgaggaagaaaaaaacaacatcaacttcaacatcgacgatctgtcctctaaactgaacgaatccatcaacaaagctatgatcaacatcaacaagttcctgaaccagtgctctgtaagctatctgatgaactccatgatcccgtacggtgttaaacgtctggaggacttcgatgcgtctctgaaagacgccctgctgaaatacatttacgacaaccgtggcactctgatcggtcaggttgatcgtctgaaggacaaagtgaacaataccttatcgaccgacatcccttttcagctcagtaaatatgtcgataaccaacgccttttgtccactctagaagcacaccatcatcaccaccatcaccatcaccat

SEQ ID NO: 4 - protein, 878 aa, Artificial Sequence
  Polypeptide Sequence of rLHN/A
MEFVNKQFNYKDPVNGVDIAYIKIPNAGQMQPVKAFKIHNKIWVIPERDTFTNPEEGDLNPPPEAKQVPVSYYDSTYLSTDNEKDNYLKGVTKLFERIYSTDLGRMLLTSIVRGIPFWGGSTIDTELKVIDTNCINVIQPDGSYRSEELNLVIIGPSADIIQFECKSFGHEVLNLTRNGYGSTQYIRFSPDFTFGFEESLEVDTNPLLGAGKFATDPAVTLAHELIHAGHRLYGIAINPNRVFKVNTNAYYEMSGLEVSFEELRTFGGHDAKFIDSLQENEFRLYYYNKFKDIASTLNKAKSIVGTTASLQYMKNVFKEKYLLSEDTSGKFSVDKLKFDKLYKMLTEIYTEDNFVKFFKVLNRKTYLNFDKAVFKINIVPKVNYTIYDGFNLRNTNLAANFNGQNTEINNMNFTKLKNFTGLFEFYKLLCVDGIITSKTKSDDDDKNKALNLQCIKVNNWDLFFSPSEDNFTNDLNKGEEITSDTNIEAAEENISLDLIQQYYLTFNFDNEPENISIENLSSDIIGQLELMPNIERFPNGKKYELDKYTMFHYLRAQEFEHGKSRIALTNSVNEALLNPSRVYTFFSSDYVKKVNKATEAAMFLGWVEQLVYDFTDETSEVSTTDKIADITIIIPYIGPALNIGNMLYKDDFVGALIFSGAVILLEFIPEIAIPVLGTFALVSYIANKVLTVQTIDNALSKRNEKWDEVYKYIVTNWLAKVNTQIDLIRKKMKEALENQAEATKAIINYQYNQYTEEEKNNINFNIDDLSSKLNESINKAMININKFLNQCSVSYLMNSMIPYGVKRLEDFDASLKDALLKYIYDNRGTLIGQVDRLKDKVNNTLSTDIPFQLSKYVDNQRLLSTLEAHHHHHHHHHH

SEQ ID NO: 5 - DNA, 1329 bp, Artificial Sequence
  Nucleotide Sequence of rL/A
atgccattcgtcaacaagcaattcaactacaaagacccagtcaacggcgtcgacatcgcatacatcaagattccgaacgccggtcaaatgcagccggttaaggcttttaagatccacaacaagatttgggttatcccggagcgtgacaccttcacgaacccggaagaaggcgatctgaacccgccaccggaagcgaagcaagtccctgtcagctactacgattcgacgtacctgagcacggataacgaaaaagataactacctgaaaggtgtgaccaagctgttcgaacgtatctacagcacggatctgggtcgcatgctgctgactagcattgttcgcggtatcccgttctggggtggtagcacgattgacaccgaactgaaggttatcgacactaactgcattaacgttattcaaccggatggtagctatcgtagcgaagagctgaatctggtcatcattggcccgagcgcagacattatccaattcgagtgcaagagctttggtcacgaggttctgaatctgacccgcaatggctatggtagcacccagtacattcgtttttcgccggattttaccttcggctttgaagagagcctggaggttgataccaatccgttgctgggtgcgggcaaattcgctaccgatccggctgtcacgctggcccatgaactgatccacgcaggccaccgcctgtacggcattgccatcaacccaaaccgtgtgttcaaggttaatacgaatgcatactacgagatgagcggcctggaagtcagcttcgaagaactgcgcaccttcggtggccatgacgctaaattcattgacagcttgcaagagaatgagttccgtctgtactactataacaaattcaaagacattgcaagcacgttgaacaaggccaaaagcatcgttggtactaccgcgtcgttgcagtatatgaagaatgtgtttaaagagaagtacctgctgtccgaggatacctccggcaagtttagcgttgataagctgaagtttgacaaactgtacaagatgctgaccgagatttacaccgaggacaactttgtgaaattcttcaaagtgttgaatcgtaaaacctatctgaattttgacaaagcggttttcaagattaacatcgtgccgaaggtgaactacaccatctatgacggttttaacctgcgtaacaccaacctggcggcgaactttaacggtcagaatacggaaatcaacaacatgaatttcacgaagttgaagaacttcacgggtctgttcgagttctataagctgctgggtctagaagcacaccatcatcaccaccatcaccatcaccat

SEQ ID NO: 6 - protein, 443 aa, Artificial Sequence
  Polypeptide Sequence of rL/A
MPFVNKQFNYKDPVNGVDIAYIKIPNAGQMQPVKAFKIHNKIWVIPERDTFTNPEEGDLNPPPEAKQVPVSYYDSTYLSTDNEKDNYLKGVTKLFERIYSTDLGRMLLTSIVRGIPFWGGSTIDTELKVIDTNCINVIQPDGSYRSEELNLVIIGPSADIIQFECKSFGHEVLNLTRNGYGSTQYIRFSPDFTFGFEESLEVDTNPLLGAGKFATDPAVTLAHELIHAGHRLYGIAINPNRVFKVNTNAYYEMSGLEVSFEELRTFGGHDAKFIDSLQENEFRLYYYNKFKDIASTLNKAKSIVGTTASLQYMKNVFKEKYLLSEDTSGKFSVDKLKFDKLYKMLTEIYTEDNFVKFFKVLNRKTYLNFDKAVFKINIVPKVNYTIYDGFNLRNTNLAANFNGQNTEINNMNFTKLKNFTGLFEFYKLLGLEAHHHHHHHHHH

SEQ ID NO: 7 - DNA, 1299 bp, Artificial Sequence
  Nucleotide Sequence of rHC/A
atgcatcatcaccatcaccacaaaaacatcatcaatactagcattctgaacctgcgttacgagagcaatcatctgattgatctgagccgttatgcaagcaagatcaacatcggtagcaaggtcaattttgacccgatcgataagaaccagatccagctgtttaatctggaatcgagcaaaattgaggttatcctgaaaaacgccattgtctacaactccatgtacgagaatttctccaccagcttctggattcgcatcccgaaatacttcaacagcattagcctgaacaacgagtatactatcatcaactgtatggagaacaacagcggttggaaggtgtctctgaactatggtgagatcatttggaccttgcaggacacccaagagatcaagcagcgcgtcgtgttcaagtactctcaaatgatcaacatttccgattacattaatcgttggatcttcgtgaccattacgaataaccgtctgaataacagcaagatttacatcaatggtcgcttgatcgatcagaaaccgattagcaacctgggtaatatccacgcaagcaacaacattatgttcaaattggacggttgccgcgatacccatcgttatatctggatcaagtatttcaacctgtttgataaagaactgaatgagaaggagatcaaagatttgtatgacaaccaatctaacagcggcattttgaaggacttctggggcgattatctgcaatacgataagccgtactatatgctgaacctgtatgatccgaacaaatatgtggatgtcaataatgtgggtattcgtggttacatgtatttgaagggtccgcgtggcagcgttatgacgaccaacatttacctgaactctagcctgtaccgtggtacgaaattcatcattaagaaatatgccagcggcaacaaagataacattgtgcgtaataacgatcgtgtctacatcaacgtggtcgtgaagaataaagagtaccgtctggcgaccaacgcttcgcaggcgggtgttgagaaaattctgagcgcgttggagatccctgatgtcggtaatctgagccaagtcgtggttatgaagagcaagaacgaccagggtatcactaacaagtgcaagatgaacctgcaagacaacaatggtaacgacatcggctttattggtttccaccagttcaacaatattgctaaactggtagcgagcaattggtacaatcgtcagattgagcgcagcagccgtactttgggctgtagctgggagtttatcccggtcgatgatggttggggcgaacgtccgctg

SEQ ID NO: 8 - protein, 433 aa, Artificial Sequence
  Polypeptide Sequence of rHC/A
MHHHHHHKNIINTSILNLRYESNHLIDLSRYASKINIGSKVNFDPIDKNQIQLFNLESSKIEVILKNAIVYNSMYENFSTSFWIRIPKYFNSISLNNEYTIINCMENNSGWKVSLNYGEIIWTLQDTQEIKQRVVFKYSQMINISDYINRWIFVTITNNRLNNSKIYINGRLIDQKPISNLGNIHASNNIMFKLDGCRDTHRYIWIKYFNLFDKELNEKEIKDLYDNQSNSGILKDFWGDYLQYDKPYYMLNLYDPNKYVDVNNVGIRGYMYLKGPRGSVMTTNIYLNSSLYRGTKFIIKKYASGNKDNIVRNNDRVYINVVVKNKEYRLATNASQAGVEKILSALEIPDVGNLSQVVVMKSKNDQGITNKCKMNLQDNNGNDIGFIGFHQFNNIAKLVASNWYNRQIERSSRTLGCSWEFIPVDDGWGERPL

SEQ ID NO: 9 - DNA, 3873 bp, Artificial Sequence
  Nucleotide Sequence of rBoNT/B(0)
atgccggtgacgattaacaacttcaactacaacgacccgattgacaacaacaacattatcatgatggaaccgccgtttgcacgcggcacgggccgttattacaaagcgtttaaaatcaccgatcgtatttggattatcccggaacgctacacgtttggttataaaccggaagacttcaacaaaagctctggcatcttcaaccgtgatgtttgcgaatactacgatccggactacctgaacaccaacgataagaaaaacatttttctgcaaacgatgatcaaactgttcaatcgcattaaaagcaaaccgctgggtgaaaaactgctggaaatgattatcaatggcattccgtatctgggtgatcgtcgcgtgccgctggaagaatttaacaccaatatcgcgagtgttacggtcaacaaactgatttccaatccgggtgaagtcgaacgtaaaaaaggcatcttcgccaacctgatcatcttcggcccgggtccggtgctgaacgaaaatgaaaccattgatatcggtattcagaaccattttgcctcacgcgaaggcttcggcggtattatgcaaatgaaattttgcccggaatatgtgtcggttttcaacaatgttcaggaaaacaaaggtgcaagcatctttaatcgtcgcggctatttctctgatccggctctgatcctgatgcaccaactgatttatgtgctgcacggcctgtatggtatcaaagtggatgacctgccgatcgttccgaacgagaaaaaatttttcatgcagagcaccgacgcaattcaagctgaagaactgtatacgtttggcggtcaggacccgtctattatcaccccgagcaccgacaaaagcatctacgataaagtgctgcaaaactttcgtggcattgttgaccgcctgaataaagtcctggtgtgtatctctgatccgaacatcaacatcaacatctacaaaaacaaattcaaagacaaatacaaattcgttgaagattctgaaggcaaatatagtattgacgtcgaatcctttgataaactgtacaaaagtctgatgttcggtttcaccgaaacgaacatcgcggaaaactacaaaatcaaaacccgcgcctcctatttcagcgactctctgccgccggttaaaatcaaaaatctgctggataacgaaatttatacgatcgaagaaggtttcaacatcagcgataaagacatggaaaaagaataccgtggccagaataaagcaatcaacaaacaggcgtatgaagaaattagtaaagaacatctggcggtctacaaaattcagatgtgcaaatccgtgaaagccccgggtatttgtatcgatgttgacaatgaagacctgtttttcatcgccgataaaaacagtttttccgatgacctgtcaaaaaatgaacgcatcgaatacaacacccaatcgaactacatcgaaaacgatttcccgatcaacgaactgattctggatacggacctgattagtaaaatcgaactgccgtcagaaaacaccgaatcgctgacggactttaatgttgatgtcccggtgtatgaaaaacagccggcaattaagaaaatttttaccgatgaaaacacgatcttccagtacctgtacagccaaacctttccgctggacattcgcgatatctctctgacgagttcctttgatgacgcactgctgttcagcaacaaagtgtactcctttttctcaatggattacatcaaaaccgctaacaaagtggttgaagcgggcctgtttgccggttgggtgaaacagatcgttaacgatttcgtcatcgaagccaacaaaagtaacacgatggataaaattgctgatatctccctgattgtcccgtatattggcctggcactgaatgtgggtaacgaaacggcgaaaggcaattttgaaaacgccttcgaaattgcaggcgcttcaatcctgctggaatttattccggaactgctgatcccggtcgtgggtgcgttcctgctggaatcttacatcgacaacaaaaacaaaatcatcaaaaccattgataacgcgctgacgaaacgtaacgaaaaatggtcagatatgtacggcctgattgttgcccagtggctgagcaccgtcaacacgcaattttacaccatcaaagaaggtatgtacaaagcgctgaattatcaggcgcaagccctggaagaaatcatcaaataccgctacaacatctacagcgaaaaagaaaaatctaacatcaacatcgactttaatgatatcaacagcaaactgaacgaaggtatcaaccaggcaatcgataacatcaacaacttcatcaacggctgctcagtgtcgtatctgatgaagaaaatgatcccgctggctgttgaaaaactgctggattttgacaacaccctgaagaaaaacctgctgaactacatcgatgaaaacaaactgtacctgatcggctcagccgaatacgaaaaatcgaaagtgaacaaatacctgaaaaccatcatgccgtttgacctgagtatttacaccaacgatacgatcctgatcgaaatgttcaacaaatacaactccgaaattctgaacaatattatcctgaacctgcgttacaaagacaacaatctgatcgatctgagcggctatggtgcaaaagttgaagtctacgacggtgtcgaactgaacgataaaaaccagttcaaactgacctcatcggctaactcaaaaattcgtgtgacgcagaaccaaaacatcatcttcaactcggtctttctggacttcagcgtgtctttctggattcgcatcccgaaatataaaaatgatggcatccagaactacatccataacgaatacaccatcatcaactgtatgaaaaacaacagtggttggaaaatttccatccgtggcaaccgcattatctggaccctgattgatatcaatggtaaaacgaaaagcgtgtttttcgaatacaacatccgtgaagatatctctgaatacatcaatcgctggtttttcgtgaccattacgaacaatctgaacaatgcgaaaatctatatcaacggcaaactggaaagtaataccgacatcaaagatattcgtgaagttatcgccaacggtgaaatcatcttcaaactggatggcgacatcgatcgcacccagttcatttggatgaaatacttctccatcttcaacacggaactgagtcagtccaatatcgaagaacgctacaaaatccaatcatactcggaatacctgaaagatttctggggtaacccgctgatgtacaacaaagaatactacatgttcaacgcgggcaacaaaaactcatacatcaaactgaaaaaagattcgccggtgggtgaaatcctgacccgtagcaaatacaaccagaactctaaatacatcaactatcgcgatctgtacattggcgaaaaatttattatccgtcgcaaaagcaactctcagagtattaatgatgacatcgtgcgtaaagaagactacatctatctggatttctttaatctgaaccaagaatggcgcgtttatacctacaaatacttcaaaaaagaagaagagaaactgttcctggccccgattagcgacagcgatgaattttacaacaccatccagatcaaagaatacgatgaacagccgacgtatagttgccaactgctgttcaaaaaagacgaagaatccaccgatgaaattggcctgattggtatccaccgtttctatgaaagcggtatcgttttcgaagaatacaaagattacttctgtatctctaaatggtatctgaaagaagtcaaacgcaaaccgtacaacctgaaactgggctgcaactggcaatttatcccgaaagacgaaggctggaccgaa

SEQ ID NO: 10 - protein, 1291 aa, Artificial Sequence
  Polypeptide Sequence of rBoNT/B(0)
MPVTINNFNYNDPIDNNNIIMMEPPFARGTGRYYKAFKITDRIWIIPERYTFGYKPEDFNKSSGIFNRDVCEYYDPDYLNTNDKKNIFLQTMIKLFNRIKSKPLGEKLLEMIINGIPYLGDRRVPLEEFNTNIASVTVNKLISNPGEVERKKGIFANLIIFGPGPVLNENETIDIGIQNHFASREGFGGIMQMKFCPEYVSVFNNVQENKGASIFNRRGYFSDPALILMHQLIYVLHGLYGIKVDDLPIVPNEKKFFMQSTDAIQAEELYTFGGQDPSIITPSTDKSIYDKVLQNFRGIVDRLNKVLVCISDPNININIYKNKFKDKYKFVEDSEGKYSIDVESFDKLYKSLMFGFTETNIAENYKIKTRASYFSDSLPPVKIKNLLDNEIYTIEEGFNISDKDMEKEYRGQNKAINKQAYEEISKEHLAVYKIQMCKSVKAPGICIDVDNEDLFFIADKNSFSDDLSKNERIEYNTQSNYIENDFPINELILDTDLISKIELPSENTESLTDFNVDVPVYEKQPAIKKIFTDENTIFQYLYSQTFPLDIRDISLTSSFDDALLFSNKVYSFFSMDYIKTANKVVEAGLFAGWVKQIVNDFVIEANKSNTMDKIADISLIVPYIGLALNVGNETAKGNFENAFEIAGASILLEFIPELLIPVVGAFLLESYIDNKNKIIKTIDNALTKRNEKWSDMYGLIVAQWLSTVNTQFYTIKEGMYKALNYQAQALEEIIKYRYNIYSEKEKSNINIDFNDINSKLNEGINQAIDNINNFINGCSVSYLMKKMIPLAVEKLLDFDNTLKKNLLNYIDENKLYLIGSAEYEKSKVNKYLKTIMPFDLSIYTNDTILIEMFNKYNSEILNNIILNLRYKDNNLIDLSGYGAKVEVYDGVELNDKNQFKLTSSANSKIRVTQNQNIIFNSVFLDFSVSFWIRIPKYKNDGIQNYIHNEYTIINCMKNNSGWKISIRGNRIIWTLIDINGKTKSVFFEYNIREDISEYINRWFFVTITNNLNNAKIYINGKLESNTDIKDIREVIANGEIIFKLDGDIDRTQFIWMKYFSIFNTELSQSNIEERYKIQSYSEYLKDFWGNPLMYNKEYYMFNAGNKNSYIKLKKDSPVGEILTRSKYNQNSKYINYRDLYIGEKFIIRRKSNSQSINDDIVRKEDYIYLDFFNLNQEWRVYTYKYFKKEEEKLFLAPISDSDEFYNTIQIKEYDEQPTYSCQLLFKKDEESTDEIGLIGIHRFYESGIVFEEYKDYFCISKWYLKEVKRKPYNLKLGCNWQFIPKDEGWTE

SEQ ID NO: 11 - DNA, 3873 bp, Artificial Sequence
  Nucleotide Sequence of rBoNT/C(0)
atgccgatcacgattaataatttcaactatagcgatccggtggacaataagaatattctgtatctggatactcatctgaatacgctggctaacgaaccggagaaagcgttccgcatcacaggcaacatctgggttattcccgatcgcttttcacgcaacagcaaccctaatctgaacaaacctcctcgtgtcaccagtcctaaatccggttattacgacccaaactatctgagtacggatagcgataaagatccctttctgaaagagatcattaagctgttcaaacgcattaactctcgcgaaattggggaagagctgatctatcggctttcgacagatatcccgttcccaggtaacaataataccccgattaatactttcgactttgatgttgatttcaattctgtggatgtgaaaacgcgtcaaggcaataattgggtgaaaactggtagcattaacccgagtgtaattatcacaggtccccgtgagaacatcatcgacccggaaacctctaccttcaagctgacgaacaacacgtttgctgcacaggaagggtttggtgccctgtcaatcatttccatctcaccgcgtttcatgttaacctactccaatgccacaaatgatgttggcgaaggacgttttagcaaatcagaattttgcatggacccaattctcattctgatgggcacgctgaacaatgcgatgcacaacttgtatggcattgctattccaaacgatcaaaccattagctccgttaccagtaatatcttctatagccagtataatgtcaaattggagtatgccgaaatttacgcctttggaggcccgaccattgacctgattccgaaatctgcacgcaaatacttcgaagaaaaggcgttagattactatcgcagcatcgcgaaacgcctgaactcgattaccacggccaatccgtcgtcgttcaacaaatacattggtgaatataaacagaaactgattcgcaaatatcggtttgtcgtagaaagctctggtgaagtgactgtaaaccgcaacaaatttgtcgaactctacaacgagttgacccaaatctttaccgagtttaactacgcaaagatctataacgtacagaaccgcaagatttatcttagcaatgtatacacaccggttactgcgaacatcttagacgacaatgtgtatgatattcagaatggctttaacatcccgaaatcaaatctgaacgttctgtttatgggccagaacctgagtcgtaatccagcactgcgtaaagtgaacccggaaaatatgctctacttgtttaccaaattttgccacaaagcgattgatggccgctctctctataacaaaacgctggattgtcgtgagttacttgtgaagaacactgatttaccgttcattggggatatctccgacgtgaaaaccgatatcttcctgcgcaaagacattaatgaagaaacggaagtcatctattaccccgacaatgtgagcgttgatcaggtcattttatcgaagaacacctccgaacatggtcagttggatttgctgtaccctagcattgactcggagagtgaaatccttccgggcgaaaatcaagtgttttacgacaaccgtacccaaaatgttgattatttgaattcttattactacctggaatctcagaaattgagcgacaatgtggaagatttcacgttcacacgctccattgaggaagcgctggataatagcgcgaaagtgtatacgtatttccctaccttggcgaataaagtaaatgctggtgtccagggaggcttatttctgatgtgggcgaatgatgtggtagaagattttacgaccaatattttgcgtaaggacaccttagataaaattagcgatgttagcgccatcatcccctatattggcccagcactgaatatctcgaactctgtgcgtcgcggaaacttcaccgaagcatttgcggtgaccggggttactattctgttggaagcctttccggagtttactattccggcgctgggtgcgtttgtgatttattcgaaagtacaagaacgcaatgaaattatcaaaaccatcgataattgcctggaacaacgcattaaacgctggaaggattcttatgaatggatgatgggcacctggttatcccgtattatcacacagtttaacaacatctcgtatcagatgtacgattcactgaactaccaagcaggggcgatcaaagccaagatcgacttagaatacaagaaatattcaggtagcgataaagagaatattaaaagccaggttgaaaacctgaagaactctctggatgtcaaaatttcagaggctatgaacaacattaacaaatttatccgcgaatgtagcgtcacgtatctgtttaaaaacatgctcccgaaagtgattgatgagctcaacgagtttgatcgcaacacaaaggccaaactgattaacctgattgatagtcacaatattattttagtcggtgaagttgacaagctgaaggctaaggtcaataacagctttcagaacactattccgtttaatattttctcctatacgaacaatagtctgctgaaagacattatcaacgaatacttcaacaatattaatgacagcaaaattctgagcctgcagaatcgtaagaatacgctggtagataccagtggatataatgcggaagtctcagaagagggtgatgtacagctgaacccgatctttccgttcgactttaaactggggtctagtggtgaagatcgcggtaaagtgatcgttacccaaaacgagaacattgtgtataacagcatgtacgagagtttctcaatttctttctggattcgcatcaataaatgggtttctaatttgcctggctataccatcattgatagcgtcaaaaacaactcgggctggtcgattggcattattagcaactttctggtgtttaccctgaaacagaatgaggattcggaacagagcattaacttctcctacgacatcagcaacaatgcaccagggtataacaaatggttcttcgtaacggtgacgaacaatatgatgggcaatatgaaaatctacattaacgggaaacttatcgacaccattaaagtgaaagagcttactgggatcaattttagtaaaaccattacctttgagatcaacaaaattccggacacgggtctgattacctccgattcggataatatcaatatgtggattcgcgacttttatatcttcgccaaagaacttgatggcaaagatatcaacattttgtttaattccctgcagtataccaatgtcgttaaggactattggggcaatgatctccgctacaataaagaatactacatggttaacatcgactatctcaatcgctacatgtatgctaactcgcgtcaaattgtgtttaacacacgtcgtaacaacaacgattttaacgaaggttataaaatcattatcaaacggatccgcggcaatacgaacgatactcgtgttcgtggcggtgacattctgtatttcgacatgacgattaataataaagcgtacaatctgttcatgaagaacgaaaccatgtacgccgataaccattccactgaagatatctacgcaatcggacttcgcgaacagaccaaagacattaacgacaacatcatctttcagattcaaccgatgaataatacctactactatgcctcccagatcttcaaaagtaatttcaacggcgaaaacatttcaggcatttgctcaatcggcacttatcggttccggttaggtggtgattggtatcgtcacaactaccttgttcccacagtgaaacaaggcaactatgcatcgctcttagaaagcacatctacgcattggggttttgtgccagtcagtgaa

SEQ ID NO: 12 - protein, 1291 aa, Artificial Sequence
  Polypeptide Sequence of rBoNT/C(0)
MPITINNFNYSDPVDNKNILYLDTHLNTLANEPEKAFRITGNIWVIPDRFSRNSNPNLNKPPRVTSPKSGYYDPNYLSTDSDKDPFLKEIIKLFKRINSREIGEELIYRLSTDIPFPGNNNTPINTFDFDVDFNSVDVKTRQGNNWVKTGSINPSVIITGPRENIIDPETSTFKLTNNTFAAQEGFGALSIISISPRFMLTYSNATNDVGEGRFSKSEFCMDPILILMGTLNNAMHNLYGIAIPNDQTISSVTSNIFYSQYNVKLEYAEIYAFGGPTIDLIPKSARKYFEEKALDYYRSIAKRLNSITTANPSSFNKYIGEYKQKLIRKYRFVVESSGEVTVNRNKFVELYNELTQIFTEFNYAKIYNVQNRKIYLSNVYTPVTANILDDNVYDIQNGFNIPKSNLNVLFMGQNLSRNPALRKVNPENMLYLFTKFCHKAIDGRSLYNKTLDCRELLVKNTDLPFIGDISDVKTDIFLRKDINEETEVIYYPDNVSVDQVILSKNTSEHGQLDLLYPSIDSESEILPGENQVFYDNRTQNVDYLNSYYYLESQKLSDNVEDFTFTRSIEEALDNSAKVYTYFPTLANKVNAGVQGGLFLMWANDVVEDFTTNILRKDTLDKISDVSAIIPYIGPALNISNSVRRGNFTEAFAVTGVTILLEAFPEFTIPALGAFVIYSKVQERNEIIKTIDNCLEQRIKRWKDSYEWMMGTWLSRIITQFNNISYQMYDSLNYQAGAIKAKIDLEYKKYSGSDKENIKSQVENLKNSLDVKISEAMNNINKFIRECSVTYLFKNMLPKVIDELNEFDRNTKAKLINLIDSHNIILVGEVDKLKAKVNNSFQNTIPFNIFSYTNNSLLKDIINEYFNNINDSKILSLQNRKNTLVDTSGYNAEVSEEGDVQLNPIFPFDFKLGSSGEDRGKVIVTQNENIVYNSMYESFSISFWIRINKWVSNLPGYTIIDSVKNNSGWSIGIISNFLVFTLKQNEDSEQSINFSYDISNNAPGYNKWFFVTVTNNMMGNMKIYINGKLIDTIKVKELTGINFSKTITFEINKIPDTGLITSDSDNINMWIRDFYIFAKELDGKDINILFNSLQYTNVVKDYWGNDLRYNKEYYMVNIDYLNRYMYANSRQIVFNTRRNNNDFNEGYKIIIKRIRGNTNDTRVRGGDILYFDMTINNKAYNLFMKNETMYADNHSTEDIYAIGLREQTKDINDNIIFQIQPMNNTYYYASQIFKSNFNGENISGICSIGTYRFRLGGDWYRHNYLVPTVKQGNYASLLESTSTHWGFVPVSE

SEQ ID NO: 13 - DNA, 3756 bp, Artificial Sequence
  Nucleotide Sequence of rBoNT/E(0)
atgccgaaaatcaactctttcaactacaacgacccggttaacgaccgtaccatcctgtatatcaaaccgggtggttgccaggagttctacaaatctttcaacatcatgaaaaacatctggatcatcccggaacgtaacgttatcggtaccaccccgcaggacttccacccgccgacctctctgaaaaacggtgactcttcttactacgacccgaactacctccagtctgacgaagaaaaagaccgtttcctgaaaatcgttaccaaaatcttcaaccgtatcaacaacaacctgtctggtggtatcctgctggaagaactgtctaaagctaacccgtacctgggtaacgacaacaccccggacaaccagttccacatcggtgacgcttctgctgttgaaatcaaattctctaacggttctcaggacatcctgctgccgaacgttatcatcatgggtgctgaaccggacctgttcgaaaccaactcttctaacatctctctgcgtaacaactacatgccgtctaaccacggtttcggttctatcgctatcgttaccttctctccggaatactctttccgtttcaacgacaacagcatgaacgagttcatccaggacccggctctgaccctgatgcaccaactgatctactctctgcacggtctgtacggtgctaaaggtatcaccaccaaatacaccatcacccagaaacagaacccgctgatcaccaacatccgtggtaccaacatcgaagagttcctgaccttcggtggtaccgacctgaacatcatcacctctgctcagtctaacgacatctacaccaacctgctggctgactacaaaaaaatcgcttctaaactgtctaaagttcaggtttctaacccgctgctgaacccgtacaaagacgttttcgaagctaaatacggtctggacaaagacgcttctggtatctactctgttaacatcaacaaattcaacgacatcttcaaaaaactgtactctttcaccgagttcgacctggcgaccaaattccaggttaaatgccgtcagacctacatcggtcagtacaaatacttcaaactgtctaacctgctgaacgactctatctacaacatctctgaaggttacaacatcaacaacctgaaagttaacttccgtggtcagaacgctaacctgaacccgcgtatcatcaccccgatcaccggtcgtggtctggttaaaaaaatcatccgtttctgcaagaatattgtaagcgttaaaggaataagaaaaagtatctgcatcgaaatcaacaacggtgaactgttcttcgttgcttctgaaaactcttacaacgacgacaacatcaacaccccgaaagaaatcgacgacaccgttacctctaacaacaactacgaaaacgacctggaccaggttatcctgaacttcaactctgaatctgctccgggtctgtctgacgaaaaactgaacctgaccatccagaacgacgcttacatcccgaaatacgactctaacggtacctctgacatcgaacagcacgacgttaacgaactgaacgttttcttctacctggacgctcagaaagttccggaaggtgaaaacaacgttaacctgacctcttctatcgacaccgctctgctggaacagccgaaaatctacaccttcttctcttctgagttcatcaacaacgttaacaaaccggttcaggctgctctgttcgtttcttggattcagcaggttctggttgacttcaccaccgaagctaaccagaaatctaccgttgacaaaatcgctgacatctctatcgttgttccgtacatcggtctggctctgaacatcggtaacgaagctcagaaaggtaacttcaaagacgctctggaactgctgggtgctggtatcctgctggagttcgaaccggaactgctgatcccgaccatcctggttttcaccatcaaatctttcctgggttcttctgacaacaaaaacaaagttatcaaagctatcaacaacgctctgaaagaacgtgacgaaaaatggaaagaagtttactctttcatcgtttctaactggatgaccaaaatcaacacccagttcaacaaacgtaaagaacagatgtaccaggctctccagaaccaggttaacgctatcaaaaccatcatcgaatctaaatacaactcttacaccctggaagaaaaaaacgaactgaccaacaaatacgacatcaaacagatcgaaaacgaactgaaccagaaagtttctatcgctatgaacaacatcgaccgtttcctgaccgaatcttctatctcttacctgatgaaactcatcaacgaagttaaaatcaacaaactgcgtgaatacgacgaaaacgttaaaacctacctgctgaactacatcatccagcacggttctatcctgggtgaatctcagcaggaactgaactctatggttaccgacaccctgaacaactctatcccgttcaaactgtcttcttacaccgacgacaaaatcctgatctcttacttcaacaaattctttaaacgcattaagagttcatcggttctgaatatgcggtacaaaaatgataaatatgtcgatacttctggatatgatagcaatatcaacattaacggcgacgtgtataaatatccgacaaataaaaaccagtttgggatatataacgacaagctgtcggaggtcaatatttctcaaaacgactatatcatttacgataataaatataaaaactttagcattagtttttgggttcgtatacctaattatgacaataaaattgtaaatgtgaataacgagtataccattataaactgtatgcgcgacaataacagtggttggaaggtatcgctgaaccataatgagattatctggaccctgcaggataatgcaggtataaaccagaaactggcttttaactatggaaacgcaaatgggatctcagattacattaataaatggatttttgttaccattacgaacgatcgcttaggcgactcaaaactttatattaatggcaatctgatagatcagaaatcaatcttaaatttgggcaatattcatgtctctgataacatcttgttcaagatcgttaattgcagttacactcgttatattggcattcgttactttaatatcttcgataaagaactggacgagacggaaatccagactctgtattcaaacgagcccaatactaatatattgaaagatttttggggtaactatcttttatatgataaagaatactatctcctgaatgtattgaagccaaacaatttcatagatagacgcaaggatagcacattaagtatcaacaatatcagatctactatactgttagcaaatcgcctctactccggtattaaagtgaagattcagcgggttaataactccagtaccaatgataatctggtccgtaagaacgatcaggtatacatcaatttcgtcgcgagcaaaactcatctcttcccgctttacgccgatacagctacgacaaacaaggaaaaaaccataaaaatttccagctccggaaacagattcaatcaagtagttgtaatgaactctgtgggtaataattgtacgatgaactttaagaataacaatgggaacaatattggacttttgggcttcaaagccgacacagtggtggcgtccacctggtattacacgcacatgcgggaccatacgaattcgaacggttgcttctggaactttatctcggaagaacacgggtggcaagaaaaa

SEQ ID NO: 14 - protein, 1252 aa, Artificial Sequence
  Polypeptide Sequence of rBoNT/E(0)
MPKINSFNYNDPVNDRTILYIKPGGCQEFYKSFNIMKNIWIIPERNVIGTTPQDFHPPTSLKNGDSSYYDPNYLQSDEEKDRFLKIVTKIFNRINNNLSGGILLEELSKANPYLGNDNTPDNQFHIGDASAVEIKFSNGSQDILLPNVIIMGAEPDLFETNSSNISLRNNYMPSNHGFGSIAIVTFSPEYSFRFNDNSMNEFIQDPALTLMHQLIYSLHGLYGAKGITTKYTITQKQNPLITNIRGTNIEEFLTFGGTDLNIITSAQSNDIYTNLLADYKKIASKLSKVQVSNPLLNPYKDVFEAKYGLDKDASGIYSVNINKFNDIFKKLYSFTEFDLATKFQVKCRQTYIGQYKYFKLSNLLNDSIYNISEGYNINNLKVNFRGQNANLNPRIITPITGRGLVKKIIRFCKNIVSVKGIRKSICIEINNGELFFVASENSYNDDNINTPKEIDDTVTSNNNYENDLDQVILNFNSESAPGLSDEKLNLTIQNDAYIPKYDSNGTSDIEQHDVNELNVFFYLDAQKVPEGENNVNLTSSIDTALLEQPKIYTFFSSEFINNVNKPVQAALFVSWIQQVLVDFTTEANQKSTVDKIADISIVVPYIGLALNIGNEAQKGNFKDALELLGAGILLEFEPELLIPTILVFTIKSFLGSSDNKNKVIKAINNALKERDEKWKEVYSFIVSNWMTKINTQFNKRKEQMYQALQNQVNAIKTIIESKYNSYTLEEKNELTNKYDIKQIENELNQKVSIAMNNIDRFLTESSISYLMKLINEVKINKLREYDENVKTYLLNYIIQHGSILGESQQELNSMVTDTLNNSIPFKLSSYTDDKILISYFNKFFKRIKSSSVLNMRYKNDKYVDTSGYDSNININGDVYKYPTNKNQFGIYNDKLSEVNISQNDYIIYDNKYKNFSISFWVRIPNYDNKIVNVNNEYTIINCMRDNNSGWKVSLNHNEIIWTLQDNAGINQKLAFNYGNANGISDYINKWIFVTITNDRLGDSKLYINGNLIDQKSILNLGNIHVSDNILFKIVNCSYTRYIGIRYFNIFDKELDETEIQTLYSNEPNTNILKDFWGNYLLYDKEYYLLNVLKPNNFIDRRKDSTLSINNIRSTILLANRLYSGIKVKIQRVNNSSTNDNLVRKNDQVYINFVASKTHLFPLYADTATTNKEKTIKISSSGNRFNQVVVMNSVGNNCTMNFKNNNGNNIGLLGFKADTVVASTWYYTHMRDHTNSNGCFWNFISEEHGWQEK

SEQ ID NO: 15 - DNA, 3834 bp, Artificial Sequence
  Nucleotide Sequence of rBoNT/F(0)
atgccggtggtcatcaacagcttcaactacaacgacccagtaaacgacgacacgatcctgtatatgcaaatcccgtatgaagagaagagcaagaagtactataaggcctttgaaatcatgcgcaatgtgtggattattccggagcgtaatacgattggtactgacccaagcgacttcgatccacctgcgtctttggaaaacggctcgtccgcatattacgacccgaattacctgaccaccgatgcggagaaagatcgttatttgaaaaccaccatcaagctgttcaaacgcattaacagcaatccggcaggtgaggtcctgctgcaagagattagctacgcaaagccttatctgggtaatgagcatacgcctattaacgagtttcacccggttacccgcactaccagcgttaacatcaagtcctcgaccaacgtgaagtctagcattatcctgaacctgctggttctgggtgccggtccggacatcttcgaaaactctagctacccggtgcgtaaactgatggatagcggcggtgtttatgacccgagcaatgacggttttggcagcatcaatatcgtgacgtttagcccggagtacgagtacaccttcaatgatatcagcggtggttacaattcttctaccgagagcttcatcgccgacccggcgatcagcctggcacaccaactgatctatgcattgcatggcttgtacggtgcccgtggtgtgacgtataaagagactatcaaggttaagcaggcacctctgatgattgcggaaaagccgattcgcctggaagagttcctgaccttcggcggtcaagatttgaacatcattacctcggccatgaaagagaaaatctataacaatttgctggccaactatgaaaagattgcaacgcgcttgtctcgtgttaactccgctccgccggaatacgacattaatgagtacaaagactactttcaatggaaatatggcctggacaaaaatgcggatggttcttataccgtgaatgaaaacaaattcaatgaaatctacaagaaactgtacagcttcaccgaaatcgatctggcgaacaagttcaaagtcaaatgtcgtaatacctacttcatcaaatatggcttcctgaaagtcccgaacctgctggacgatgacatctataccgtcagcgaaggcttcaacatcggcaatctggccgtgaataatcgtggtcagaacatcaaactgaatccgaaaatcattgactccatcccagacaagggcctggttgagaaaatcgtgaagttctgcaaaagcgttattccgcgtaaaggtacgaaagcaccgcctcgcctgtgcattcgcgttaacaaccgtgagttgttctttgtggcatctgaaagcagctacaacgagaacgacatcaacacccctaaagaaattgatgataccacgaacctgaataacaattatcgcaacaatctggacgaggtgatcctggattacaattcggaaaccattccgcaaattagcaatcagacgctgaacaccctggttcaggacgatagctacgttccgcgttacgactccaatggtactagcgagattgaagaacacaacgtagtggacttgaacgttttcttttatctgcacgcccagaaggttccggagggcgaaaccaatattagcctgaccagctcgatcgacaccgcgctgtctgaggagagccaagtctacacctttttcagcagcgagtttatcaacactattaacaagccagttcatgctgcattgtttatctcttggattaaccaggtgattcgcgactttacgacggaggcgacccagaagtctaccttcgacaaaattgcagacatctccctggtcgtcccatacgtcggcctggcgttgaatattggcaatgaagttcaaaaagagaacttcaaagaagcgttcgagctgctgggtgcaggcatcctgctggagttcgtgccggaactgttgatcccgaccatcctggtgttcaccattaagagcttcattggatcctccgagaataagaacaagatcatcaaggcgatcaataacagcctgatggagcgtgaaacgaagtggaaagaaatctatagctggattgttagcaattggctgactcgtattaacacgcaattcaacaagcgtaaagagcaaatgtaccaagccctgcaaaaccaagttgacgccatcaaaacggtaattgaatacaagtacaacaattacacgagcgatgagcgcaaccgcctggaaagcgaatacaacatcaacaacattcgcgaagaattgaacaagaaagtgagcctggcgatggagaacattgagcgttttatcaccgaaagcagcatcttttacctgatgaaattgattaatgaggcgaaagtctcgaaactgcgtgagtacgacgaaggtgtgaaagagtatctgctggattacattagcgagcaccgtagcatcttgggtaactcggttcaggagctgaacgatctggtgacctctaccctgaacaatagcatcccgttcgaactgagcagctataccaatgacaagattctgattctgtatttcaataaactgtataagaagatcaaggataacagcattctggatatgcgttacgaaaacaataagtttatcgacatttctggttacggcagcaacatttccatcaatggcgatgtctacatctacagcaccaatcgcaaccagttcggcatctactctagcaaaccgagcgaagttaacatcgcacagaacaatgatattatttataacggtcgttatcaaaacttctctatcagcttttgggtccgtatcccgaagtacttcaataaagtcaatctgaataatgaatacacgatcatcgactgcattcgcaataacaacagcggttggaaaatcagcctgaattacaacaaaattatttggaccctgcaagatacggcgggtaacaatcagaaactggtgtttaactacacgcaaatgatcagcatttctgactatatcaacaagtggatctttgttaccatcaccaataatcgtctgggcaatagccgtatttacatcaacggtaacctgattgatgagaaaagcatcagcaacctgggcgatattcacgtcagcgacaacattctgttcaaaattgttggttgtaacgatacccgttacgtcggcatccgttatttcaaggttttcgatacggagctgggtaaaacggaaatcgaaacgttgtactccgatgaaccagatccgagcattctgaaggacttttggggtaactacttgctgtacaataaacgttactatctgctgaatctgttgcgcaccgacaagagcattacccaaaacagcaatttcctgaacattaatcagcaacgcggcgtataccaaaaaccgaacatcttcagcaatacgcgcctgtatactggtgttgaagtgatcattcgtaagaacggtagcaccgacattagcaacacggacaatttcgtccgtaagaatgacctggcgtacattaacgtcgtggaccgtgatgtcgagtatcgtctgtacgcagacatcagcattgcgaaaccggaaaagattatcaagctgatccgtaccagcaacagcaacaacagcctgggtcagatcattgtgatggacagcattggtaataactgcacgatgaacttccagaacaacaatggtggtaatatcggtctgctgggttttcacagcaataatctggttgcttccagctggtactacaataacattcgtaaaaacacgtctagcaatggttgtttttggagctttatcagcaaagagcacggctggcaagaaaat

SEQ ID NO: 16 - protein, 1278 aa, Artificial Sequence
  Polypeptide Sequence of rBoNT/F(0)
MPVVINSFNYNDPVNDDTILYMQIPYEEKSKKYYKAFEIMRNVWIIPERNTIGTDPSDFDPPASLENGSSAYYDPNYLTTDAEKDRYLKTTIKLFKRINSNPAGEVLLQEISYAKPYLGNEHTPINEFHPVTRTTSVNIKSSTNVKSSIILNLLVLGAGPDIFENSSYPVRKLMDSGGVYDPSNDGFGSINIVTFSPEYEYTFNDISGGYNSSTESFIADPAISLAHQLIYALHGLYGARGVTYKETIKVKQAPLMIAEKPIRLEEFLTFGGQDLNIITSAMKEKIYNNLLANYEKIATRLSRVNSAPPEYDINEYKDYFQWKYGLDKNADGSYTVNENKFNEIYKKLYSFTEIDLANKFKVKCRNTYFIKYGFLKVPNLLDDDIYTVSEGFNIGNLAVNNRGQNIKLNPKIIDSIPDKGLVEKIVKFCKSVIPRKGTKAPPRLCIRVNNRELFFVASESSYNENDINTPKEIDDTTNLNNNYRNNLDEVILDYNSETIPQISNQTLNTLVQDDSYVPRYDSNGTSEIEEHNVVDLNVFFYLHAQKVPEGETNISLTSSIDTALSEESQVYTFFSSEFINTINKPVHAALFISWINQVIRDFTTEATQKSTFDKIADISLVVPYVGLALNIGNEVQKENFKEAFELLGAGILLEFVPELLIPTILVFTIKSFIGSSENKNKIIKAINNSLMERETKWKEIYSWIVSNWLTRINTQFNKRKEQMYQALQNQVDAIKTVIEYKYNNYTSDERNRLESEYNINNIREELNKKVSLAMENIERFITESSIFYLMKLINEAKVSKLREYDEGVKEYLLDYISEHRSILGNSVQELNDLVTSTLNNSIPFELSSYTNDKILILYFNKLYKKIKDNSILDMRYENNKFIDISGYGSNISINGDVYIYSTNRNQFGIYSSKPSEVNIAQNNDIIYNGRYQNFSISFWVRIPKYFNKVNLNNEYTIIDCIRNNNSGWKISLNYNKIIWTLQDTAGNNQKLVFNYTQMISISDYINKWIFVTITNNRLGNSRIYINGNLIDEKSISNLGDIHVSDNILFKIVGCNDTRYVGIRYFKVFDTELGKTEIETLYSDEPDPSILKDFWGNYLLYNKRYYLLNLLRTDKSITQNSNFLNINQQRGVYQKPNIFSNTRLYTGVEVIIRKNGSTDISNTDNFVRKNDLAYINVVDRDVEYRLYADISIAKPEKIIKLIRTSNSNNSLGQIIVMDSIGNNCTMNFQNNNGGNIGLLGFHSNNLVASSWYYNNIRKNTSSNGCFWSFISKEHGWQEN

SEQ ID NO: 17 - DNA, 3942 bp, Artificial Sequence
  Nucleotide Sequence of rBoNT/A(0) (His-tagged)
atgccgtttgtgaacaagcagttcaactataaagatccggttaatggtgtggatatcgcctatatcaaaattccgaatgcaggtcagatgcagccggttaaagcctttaaaatccataacaaaatttgggtgattccggaacgtgatacctttaccaatccggaagaaggtgatctgaatccgcctccggaagcaaaacaggttccggttagctattatgatagcacctatctgagcaccgataacgagaaagataactatctgaaaggtgtgaccaaactgtttgaacgcatttatagtaccgatctgggtcgtatgctgctgaccagcattgttcgtggtattccgttttggggtggtagcaccattgataccgaactgaaagttattgacaccaactgcattaatgtgattcagccggatggtagctatcgtagcgaagaactgaatctggttattattggtccgagcgcagatatcattcagtttgaatgtaaaagctttggccacgaagttctgaatctgacccgtaatggttatggtagtacccagtatattcgtttcagtccggattttacctttggctttgaagaaagcctggaagttgatacaaatccgctgttaggtgcaggtaaatttgcaaccgatccggcagttaccctggcacaccagctgatttatgccggtcatcgtctgtatggtattgccattaatccgaatcgtgtgttcaaagtgaataccaacgcctattatgaaatgagcggtctggaagtgagttttgaagaactgcgtacctttggtggtcatgatgccaaatttatcgatagcctgcaagaaaatgaatttcgcctgtactactataacaaattcaaggatattgcgagcaccctgaataaagccaaaagcattgttggcaccaccgcaagcctgcagtatatgaaaaatgtgtttaaagaaaaatatctgctgagcgaagataccagcggtaaatttagcgttgacaaactgaaattcgataaactgtacaagatgctgaccgagatttataccgaagataacttcgtgaagtttttcaaagtgctgaaccgcaaaacctacctgaactttgataaagccgtgttcaaaatcaacatcgtgccgaaagtgaactataccatctatgatggttttaacctgcgcaataccaatctggcagcaaactttaatggtcagaacaccgaaatcaacaacatgaactttaccaaactgaagaacttcaccggtctgttcgaattttacaaactgctgtgtgttcgtggcattattaccagcaaaaccaaaagtctggataaaggctacaataaagccctgaatgatctgtgcattaaggtgaataattgggacctgttttttagcccgagcgaggataatttcaccaacgatctgaacaaaggcgaagaaattaccagcgataccaatattgaagcagccgaagaaaacattagcctggatctgattcagcagtattatctgaccttcaacttcgataatgagccggaaaatatcagcattgaaaacctgagcagcgatattattggccagctggaactgatgccgaatattgaacgttttccgaacggcaaaaaatacgagctggataaatacaccatgttccattatctgcgtgcccaagaatttgaacatggtaaaagccgtattgcactgaccaatagcgttaatgaagcactgctgaacccgagccgtgtttataccttttttagcagcgattacgtgaaaaaggttaacaaagcaaccgaagcagccatgtttttaggttgggttgaacagctggtttatgatttcaccgatgaaaccagcgaagttagcaccaccgataaaattgcagatattaccatcatcatcccgtatatcggtccggcactgaatattggcaatatgctgtataaagacgattttgtgggtgccctgatttttagcggtgcagttattctgctggaatttattccggaaattgccattccggttctgggcacctttgcactggtgagctatattgcaaataaagttctgaccgtgcagaccatcgataatgcactgagcaaacgtaacgaaaaatgggatgaagtgtacaagtatatcgtgaccaattggctggcaaaagttaacacccagattgacctgattcgcaagaagatgaaagaagcactggaaaatcaggcagaagcaaccaaagccattatcaactatcagtataaccagtacaccgaagaagagaaaaataacatcaacttcaacatcgacgatctgtccagcaaactgaacgaaagcatcaacaaagccatgattaacattaacaaatttctgaaccagtgcagcgtgagctatctgatgaatagcatgattccgtatggtgtgaaacgtctggaagattttgatgcaagcctgaaagatgccctgctgaaatatatctatgataatcgtggcaccctgattggtcaggttgatcgtctgaaagataaagtgaacaacaccctgagtaccgatattccttttcagctgagcaaatatgtggataatcagcgtctgctgtcaacctttaccgaatacattaagaacatcatcaacaccagcattctgaacctgcgttatgaaagcaatcatctgattgatctgagccgttatgccagcaaaatcaatataggcagcaaggttaacttcgacccgattgacaaaaatcagatacagctgtttaatctggaaagcagcaaaattgaggtgatcctgaaaaacgccattgtgtataatagcatgtacgagaatttctcgaccagcttttggattcgtatcccgaaatactttaatagcatcagcctgaacaacgagtacaccattattaactgcatggaaaacaatagcggctggaaagttagcctgaattatggcgaaattatctggaccctgcaggatacccaagaaatcaaacagcgtgtggttttcaaatacagccagatgattaatatcagcgactatatcaaccgctggatttttgtgaccattaccaataatcgcctgaataacagcaagatctatattaacggtcgtctgattgaccagaaaccgattagtaatctgggtaatattcatgcgagcaacaacatcatgtttaaactggatggttgtcgtgatacccatcgttatatttggatcaagtacttcaacctgttcgataaagagttgaacgaaaaagaaattaaagacctgtatgataaccagagcaacagcggtattctgaaggatttttggggagattatctgcagtatgacaaaccgtattatatgctgaatctgtacgacccgaataaatacgtggatgtgaataatgttggcatccgtggttatatgtacctgaaaggtccgcgtggtagcgttatgaccacaaacatttatctgaatagcagcctgtatcgcggaaccaaattcatcattaaaaagtatgccagcggcaacaaggataatattgtgcgtaataatgatcgcgtgtacattaacgttgtggtgaagaataaagaatatcgcctggcaaccaatgcaagccaggcaggcgttgaaaaaattctgagtgccctggaaattccggatgttggtaatctgagccaggttgttgtgatgaaaagcaaaaatgatcagggcatcaccaacaagtgcaaaatgaatctgcaggacaataacggcaacgatattggttttattggcttccaccagttcaacaatattgcgaaactggttgcaagcaattggtataatcgtcagattgaacgtagcagtcgtaccctgggttgtagctgggaatttatccctgtggatgatggttggggtgaacgtccgctggaaaacctgtattttcaaggtgcaagtcatcatcaccatcaccaccatcattaa

SEQ ID NO: 18 - protein, 1313 aa, Artificial Sequence
  Polypeptide Sequence of rBoNT/A(0) (His-tagged)
MPFVNKQFNYKDPVNGVDIAYIKIPNAGQMQPVKAFKIHNKIWVIPERDTFTNPEEGDLNPPPEAKQVPVSYYDSTYLSTDNEKDNYLKGVTKLFERIYSTDLGRMLLTSIVRGIPFWGGSTIDTELKVIDTNCINVIQPDGSYRSEELNLVIIGPSADIIQFECKSFGHEVLNLTRNGYGSTQYIRFSPDFTFGFEESLEVDTNPLLGAGKFATDPAVTLAHQLIYAGHRLYGIAINPNRVFKVNTNAYYEMSGLEVSFEELRTFGGHDAKFIDSLQENEFRLYYYNKFKDIASTLNKAKSIVGTTASLQYMKNVFKEKYLLSEDTSGKFSVDKLKFDKLYKMLTEIYTEDNFVKFFKVLNRKTYLNFDKAVFKINIVPKVNYTIYDGFNLRNTNLAANFNGQNTEINNMNFTKLKNFTGLFEFYKLLCVRGIITSKTKSLDKGYNKALNDLCIKVNNWDLFFSPSEDNFTNDLNKGEEITSDTNIEAAEENISLDLIQQYYLTFNFDNEPENISIENLSSDIIGQLELMPNIERFPNGKKYELDKYTMFHYLRAQEFEHGKSRIALTNSVNEALLNPSRVYTFFSSDYVKKVNKATEAAMFLGWVEQLVYDFTDETSEVSTTDKIADITIIIPYIGPALNIGNMLYKDDFVGALIFSGAVILLEFIPEIAIPVLGTFALVSYIANKVLTVQTIDNALSKRNEKWDEVYKYIVTNWLAKVNTQIDLIRKKMKEALENQAEATKAIINYQYNQYTEEEKNNINFNIDDLSSKLNESINKAMININKFLNQCSVSYLMNSMIPYGVKRLEDFDASLKDALLKYIYDNRGTLIGQVDRLKDKVNNTLSTDIPFQLSKYVDNQRLLSTFTEYIKNIINTSILNLRYESNHLIDLSRYASKINIGSKVNFDPIDKNQIQLFNLESSKIEVILKNAIVYNSMYENFSTSFWIRIPKYFNSISLNNEYTIINCMENNSGWKVSLNYGEIIWTLQDTQEIKQRVVFKYSQMINISDYINRWIFVTITNNRLNNSKIYINGRLIDQKPISNLGNIHASNNIMFKLDGCRDTHRYIWIKYFNLFDKELNEKEIKDLYDNQSNSGILKDFWGDYLQYDKPYYMLNLYDPNKYVDVNNVGIRGYMYLKGPRGSVMTTNIYLNSSLYRGTKFIIKKYASGNKDNIVRNNDRVYINVVVKNKEYRLATNASQAGVEKILSALEIPDVGNLSQVVVMKSKNDQGITNKCKMNLQDNNGNDIGFIGFHQFNNIAKLVASNWYNRQIERSSRTLGCSWEFIPVDDGWGERPLENLYFQGASHHHHHHHH

SEQ ID NO: 19 - DNA, 2649 bp, Artificial Sequence
  Nucleotide Sequence of rLHN/A (His-tagged)
atgccgtttgtgaacaagcagttcaactataaagatccggttaatggtgtggatatcgcctatatcaaaattccgaatgcaggtcagatgcagccggttaaagcctttaaaatccataacaaaatttgggtgattccggaacgtgatacctttaccaatccggaagaaggtgatctgaatccgcctccggaagcaaaacaggttccggttagctattatgatagcacctatctgagcaccgataacgagaaagataactatctgaaaggtgtgaccaaactgtttgaacgcatttatagtaccgatctgggtcgtatgctgctgaccagcattgttcgtggtattccgttttggggtggtagcaccattgataccgaactgaaagttattgacaccaactgcattaatgtgattcagccggatggtagctatcgtagcgaagaactgaatctggttattattggtccgagcgcagatatcattcagtttgaatgtaaatcctttggccacgaagttctgaatctgacccgtaatggttatggtagtacccagtatattcgtttcagtccggattttacctttggctttgaagaaagcctggaagttgatacaaatccgctgttaggtgcaggtaaatttgcaaccgatccggcagttaccctggcacatgaactgattcatgccggtcatcgtctgtatggtattgcaattaatccgaaccgtgtgttcaaagtgaataccaacgcatattatgaaatgagcggtctggaagtgtcatttgaagaactgcgtacctttggtggtcatgatgccaaatttatcgatagcctgcaagaaaatgaatttcgcctgtactactataacaaattcaaggatattgcgagcaccctgaataaagccaaaagcattgttggcaccaccgcaagcctgcagtatatgaaaaatgtgtttaaagaaaaatatctgctgagcgaagataccagcggtaaatttagcgttgacaaactgaaattcgataaactgtacaagatgctgaccgagatttataccgaagataacttcgtgaagtttttcaaagtgctgaaccgcaaaacctacctgaactttgataaagccgtgttcaaaatcaacatcgtgccgaaagtgaactataccatctatgatggttttaacctgcgcaataccaatctggcagcaaactttaatggtcagaacaccgaaatcaacaacatgaactttaccaaactgaagaacttcaccggtctgttcgaattttacaaactgctgtgtgttcgtggcattattaccagcaaaaccaaaagtctggataaaggctacaataaagccctgaatgatctgtgcattaaggtgaataattgggacctgttttttagcccgagcgaggataatttcaccaacgatctgaacaaaggcgaagaaattaccagcgataccaatattgaagcagccgaagaaaacattagcctggatctgattcagcagtattatctgaccttcaacttcgataatgagccggaaaatatcagcattgaaaacctgagcagcgatattattggccagctggaactgatgccgaatattgaacgttttccgaacggcaaaaaatacgagctggataaatacaccatgttccattatctgcgtgcccaagaatttgaacatggtaaaagccgtattgcactgaccaatagcgttaatgaagcactgctgaacccgagccgtgtttataccttttttagcagcgattacgtgaaaaaggttaacaaagcaaccgaagcagccatgtttttaggttgggttgaacagctggtttatgatttcaccgatgaaaccagcgaagttagcaccaccgataaaattgcagatattaccatcatcatcccgtatatcggtccggcactgaatattggcaatatgctgtataaagacgattttgtgggtgccctgatttttagcggtgcagttattctgctggaatttattccggaaattgccattccggttctgggcacctttgcactggtgagctatattgcaaataaagttctgaccgtgcagaccatcgataatgcactgagcaaacgtaacgaaaaatgggatgaagtgtacaagtatatcgtgaccaattggctggcaaaagttaacacccagattgacctgattcgcaagaagatgaaagaagcactggaaaatcaggcagaagcaaccaaagccattatcaactatcagtataaccagtacaccgaagaagagaaaaataacatcaacttcaacatcgacgatctgtccagcaaactgaacgaaagcatcaacaaagccatgattaacattaacaaatttctgaaccagtgcagcgtgagctatctgatgaatagcatgattccgtatggtgtgaaacgtctggaagattttgatgcaagcctgaaagatgccctgctgaaatatatctatgataatcgtggcaccctgattggtcaggttgatcgtctgaaagataaagtgaacaacaccctgagtaccgatattccttttcagctgagcaaatatgtggataatcagcgtctgctgtcaaccgaaaatctgtatttccagggtgcaagtcatcatcaccatcaccaccatcattaa

SEQ ID NO: 20 - protein, 882 aa, Artificial Sequence
  Polypeptide Sequence of rLHN/A (His-tagged)
MPFVNKQFNYKDPVNGVDIAYIKIPNAGQMQPVKAFKIHNKIWVIPERDTFTNPEEGDLNPPPEAKQVPVSYYDSTYLSTDNEKDNYLKGVTKLFERIYSTDLGRMLLTSIVRGIPFWGGSTIDTELKVIDTNCINVIQPDGSYRSEELNLVIIGPSADIIQFECKSFGHEVLNLTRNGYGSTQYIRFSPDFTFGFEESLEVDTNPLLGAGKFATDPAVTLAHELIHAGHRLYGIAINPNRVFKVNTNAYYEMSGLEVSFEELRTFGGHDAKFIDSLQENEFRLYYYNKFKDIASTLNKAKSIVGTTASLQYMKNVFKEKYLLSEDTSGKFSVDKLKFDKLYKMLTEIYTEDNFVKFFKVLNRKTYLNFDKAVFKINIVPKVNYTIYDGFNLRNTNLAANFNGQNTEINNMNFTKLKNFTGLFEFYKLLCVRGIITSKTKSLDKGYNKALNDLCIKVNNWDLFFSPSEDNFTNDLNKGEEITSDTNIEAAEENISLDLIQQYYLTFNFDNEPENISIENLSSDIIGQLELMPNIERFPNGKKYELDKYTMFHYLRAQEFEHGKSRIALTNSVNEALLNPSRVYTFFSSDYVKKVNKATEAAMFLGWVEQLVYDFTDETSEVSTTDKIADITIIIPYIGPALNIGNMLYKDDFVGALIFSGAVILLEFIPEIAIPVLGTFALVSYIANKVLTVQTIDNALSKRNEKWDEVYKYIVTNWLAKVNTQIDLIRKKMKEALENQAEATKAIINYQYNQYTEEEKNNINFNIDDLSSKLNESINKAMININKFLNQCSVSYLMNSMIPYGVKRLEDFDASLKDALLKYIYDNRGTLIGQVDRLKDKVNNTLSTDIPFQLSKYVDNQRLLSTENLYFQGASHHHHHHHH

SEQ ID NO: 21 - DNA, 1323 bp, Artificial Sequence
  Nucleotide Sequence of rHC/A (His-tagged)
atgcatcatcaccatcaccacgaaaatctatacttccaaggaaaaaacatcatcaatactagcattctgaacctgcgttacgagagcaatcatctgattgatctgagccgttatgcaagcaagatcaacatcggtagcaaggtcaattttgacccgatcgataagaaccagatccagctgtttaatctggaatcgagcaaaattgaggttatcctgaaaaacgccattgtctacaactccatgtacgagaatttctccaccagcttctggattcgcatcccgaaatacttcaacagcattagcctgaacaacgagtatactatcatcaactgtatggagaacaacagcggttggaaggtgtctctgaactatggtgagatcatttggaccttgcaggacacccaagagatcaagcagcgcgtcgtgttcaagtactctcaaatgatcaacatttccgattacattaatcgttggatcttcgtgaccattacgaataaccgtctgaataacagcaagatttacatcaatggtcgcttgatcgatcagaaaccgattagcaacctgggtaatatccacgcaagcaacaacattatgttcaaattggacggttgccgcgatacccatcgttatatctggatcaagtatttcaacctgtttgataaagaactgaatgagaaggagatcaaagatttgtatgacaaccaatctaacagcggcattttgaaggacttctggggcgattatctgcaatacgataagccgtactatatgctgaacctgtatgatccgaacaaatatgtggatgtcaataatgtgggtattcgtggttacatgtatttgaagggtccgcgtggcagcgttatgacgaccaacatttacctgaactctagcctgtaccgtggtacgaaattcatcattaagaaatatgccagcggcaacaaagataacattgtgcgtaataacgatcgtgtctacatcaacgtggtcgtgaagaataaagagtaccgtctggcgaccaacgcttcgcaggcgggtgttgagaaaattctgagcgcgttggagatccctgatgtcggtaatctgagccaagtcgtggttatgaagagcaagaacgaccagggtatcactaacaagtgcaagatgaacctgcaagacaacaatggtaacgacatcggctttattggtttccaccagttcaacaatattgctaaactggtagcgagcaattggtacaatcgtcagattgagcgcagcagccgtactttgggctgtagctgggagtttatcccggtcgatgatggttggggcgaacgtccgctgtaa

SEQ ID NO: 22 - protein, 440 aa, Artificial Sequence
  Polypeptide Sequence of rHC/A (His-tagged)
MHHHHHHENLYFQGKNIINTSILNLRYESNHLIDLSRYASKINIGSKVNFDPIDKNQIQLFNLESSKIEVILKNAIVYNSMYENFSTSFWIRIPKYFNSISLNNEYTIINCMENNSGWKVSLNYGEIIWTLQDTQEIKQRVVFKYSQMINISDYINRWIFVTITNNRLNNSKIYINGRLIDQKPISNLGNIHASNNIMFKLDGCRDTHRYIWIKYFNLFDKELNEKEIKDLYDNQSNSGILKDFWGDYLQYDKPYYMLNLYDPNKYVDVNNVGIRGYMYLKGPRGSVMTTNIYLNSSLYRGTKFIIKKYASGNKDNIVRNNDRVYINVVVKNKEYRLATNASQAGVEKILSALEIPDVGNLSQVVVMKSKNDQGITNKCKMNLQDNNGNDIGFIGFHQFNNIAKLVASNWYNRQIERSSRTLGCSWEFIPVDDGWGERPL

SEQ ID NO: 23 - DNA, 1326 bp, Artificial Sequence
  Nucleotide Sequence of rLC/A (His-tagged)
atgccgtttgtgaacaagcagttcaactataaagatccggttaatggtgtggatatcgcctatatcaaaattccgaatgcaggtcagatgcagccggttaaagcctttaaaatccataacaaaatttgggtgattccggaacgtgatacctttaccaatccggaagaaggtgatctgaatccgcctccggaagcaaaacaggttccggttagctattatgatagcacctatctgagcaccgataacgagaaagataactatctgaaaggtgtgaccaaactgtttgaacgcatttatagtaccgatctgggtcgtatgctgctgaccagcattgttcgtggtattccgttttggggtggtagcaccattgataccgaactgaaagttattgacaccaactgcattaatgtgattcagccggatggtagctatcgtagcgaagaactgaatctggttattattggtccgagcgcagatatcattcagtttgaatgtaaatcctttggccacgaagttctgaatctgacccgtaatggttatggtagtacccagtatattcgtttcagtccggattttacctttggctttgaagaaagcctggaagttgatacaaatccgctgttaggtgcaggtaaatttgcaaccgatccggcagttaccctggcacatgaactgattcatgccggtcatcgtctgtatggtattgcaattaatccgaaccgtgtgttcaaagtgaataccaacgcatattatgaaatgagcggtctggaagtgtcatttgaagaactgcgtacctttggtggtcatgatgccaaatttatcgatagcctgcaagaaaatgaatttcgcctgtactactataacaaattcaaggatattgcgagcaccctgaataaagccaaaagcattgttggcaccaccgcaagcctgcagtatatgaaaaatgtgtttaaagaaaaatatctgctgagcgaagataccagcggtaaatttagcgttgacaaactgaaattcgataaactgtacaagatgctgaccgagatttataccgaagataacttcgtgaagtttttcaaagtgctgaaccgcaaaacctacctgaactttgataaagccgtgttcaaaatcaacatcgtgccgaaagtgaactataccatctatgatggttttaacctgcgcaataccaatctggcagcaaactttaatggtcagaacaccgaaatcaacaacatgaactttaccaaactgaagaacttcaccggtctgtttgaagagaatctgtatttccagggtgcaagtcatcatcaccatcaccaccatcattaa

SEQ ID NO: 24 - protein, 441 aa, Artificial Sequence
  Polypeptide Sequence of rLC/A (His-tagged)
MPFVNKQFNYKDPVNGVDIAYIKIPNAGQMQPVKAFKIHNKIWVIPERDTFTNPEEGDLNPPPEAKQVPVSYYDSTYLSTDNEKDNYLKGVTKLFERIYSTDLGRMLLTSIVRGIPFWGGSTIDTELKVIDTNCINVIQPDGSYRSEELNLVIIGPSADIIQFECKSFGHEVLNLTRNGYGSTQYIRFSPDFTFGFEESLEVDTNPLLGAGKFATDPAVTLAHELIHAGHRLYGIAINPNRVFKVNTNAYYEMSGLEVSFEELRTFGGHDAKFIDSLQENEFRLYYYNKFKDIASTLNKAKSIVGTTASLQYMKNVFKEKYLLSEDTSGKFSVDKLKFDKLYKMLTEIYTEDNFVKFFKVLNRKTYLNFDKAVFKINIVPKVNYTIYDGFNLRNTNLAANFNGQNTEINNMNFTKLKNFTGLFEENLYFQGASHHHHHHHH

SEQ ID NO: 25 - DNA, 3918 bp, Artificial Sequence
  Nucleotide Sequence of rBoNT/FA(0) (His-tagged)
atgccggttgtgattaacagcttcaattatgatgatccggtgaacgataacaccatcatttatatccgtccgccttattatgaaaccagcaacacctatttcaaagccttccagattatggataacgtgtggattattccggaacgttatcgtctgggtattgatccgagcctgtttaatccgcctgttagcctgaaagcaggtagtgatggttattttgatccgaattatctgagcaccaacaccgagaaaaacaaatacctgcagattatgatcaagctgttcaaacgcattaatagcaaaccggcaggtcagattctgctggaagaaatcaaaaatgcaattccgtatctgggcaacagctatacccaagaagaacagtttaccaccaataatcgtaccgtgagctttaatgttaaactggccaatggtaatatcgttcagcagatggcaaatctgattatttggggtccgggtcctgatctgaccacaaataaaaccggtggtatcatctatagcccgtatcagagcatggaagcaaccccgtataaagatggttttggtagcattatgaccgtggaatttagtccggaatatgcaaccgcctttaacgatatttcaattgcaagccatagtccgtcgctgtttatcaaagatccggcactgattctgatgcaccagctgatttatgttctgcatggtctgtatggcacctatatcaccgaatacaaaattaccccgaatgtggttcagagctatatgaaagttaccaaaccgattaccagcgcagaatttctgacctttggtggtcgtgatcgcaatattgttccgcagagcattcagagccagctgtataacaaagttctgagcgattataaacgtattgccagccgtctgaataaagttaataccgcaaccgcactgatcaacatcgatgaattcaaaaacctgtacgagtggaaataccagtttgccaaagatagcaatggtgtgtatagcgtggatctgaacaaatttgagcagctgtacaaaaaaatctatagcttcaccgaattcaacctggcctatgagtttaaaatcaaaacccgtctgggttatctggccgaaaattttggtccgttttatctgccgaatctgctggatgatagcatttataccgaagtggatggttttaacattggtgcactgagcattaactatcagggtcagaatattggcagcgatatcaacagcatcaaaaaactgcaaggtcagggtgttgttagccgtgttgttcgtctgtgtagcaatagcaataccaaaaacagcctgtgcattaccgttaataatcgcgacctgttttttatcgcaagccaagaaagctatggcgagaataccattaacacctataaagagattgacgataccaccacactggatccgagctttgaagatattctggataaagtgatcctgaacttcaacgaacaggttattccgcagatgccgaatcgtaatgttagcaccgatattcagaaagacaactacatcccgaaatacgattataaccgcaccgacattatcgatagctatgaagttggtcgcaactacaacacctttttctatctgaatgcccagaaatttagcccgaacgaaagcaatattaccctgaccagcagctttgatacaggtctgttagaaggtagcaaagtgtatacctttttcagcagcgatttcattaacaacatcaacaaaccggttcaggccctgctgtttattgaatgggttaaacaggtgattcgcgattttaccaccgaagcaaccaaaacctcaaccgttgataaactgaaagatattagcctggtggtgccgtatattggtctggcactgaatattggtgatgagatctacaaacagcattttgcagaagcagttgaactggttggtgcaggtctgctgctggaattttcaccggaatttcttattccgacgctgctgatttttaccatcaaaggttatctgaccggtagcattcgcgataaagacaaaatcattaaaaccctggataacgccctgaatgttcgtgatcagaaatggaaagaactgtatcgttgggttgttagcaaatggctgaccaccattaatacgcagttcaacaaacgcaaagaacaaatgtacaaagccctgaaaaatcaggccaccgccattaaaaagatcatcgagaacaaatataacaactataccaccgatgaaaaaagcaagatcgatagcagctataacatcaacgaaattgaacgcaccctgaacgaaaaaatcaatctggccatgaaaaacatcgagcagtttattaccgaaagcagcattgcctatctgatcaatatcatcaacaacgaaacgatccagaaactgaaaagctatgatgacctggttcgtcgttatctgctgggttatattcgtaatcatagcagcattctgggcaatagcgttgaagaactgaattccaaagtgaacaaccatctggataatggcattccgtttgaactgagcagttataccaatgatagcctgctgatccgctacttcaataaaaactatggcgaactgaagtacaactgcattctgaacatcaaatatgagatggatcgtgacaaactggttgatagcagcggttatcgtagccgtatcaatattggtacaggcgtcaaatttagcgagatcgataaaaatcaagtgcagctgagcaatctggaatccagcaaaattgaagtcattctgaataacggcgtcatctataacagcatgtatgaaaacttttcgaccagcttttggattcgcattccgaaatactttcgcaacatcaataacgagtacaagatcatcagctgtatgcagaataatagcggttgggaagtgagcctgaattttagcaatatgaactcgaaaatcatctggaccctgcaggataccgaaggtatcaaaaaaaccgttgtgtttcagtacacccagaacattaacattagcgactatatcaaccgctggatctttgtgaccattacaaataatcgtctgagcaacagcaaaatctacattaatggtcgcctgatcaacgaagaaagcattagcgatctgggtaatatccatgccagcaacaacattatgtttaaactggatggttgccgtgatccgcatcgttatatctggattaaatactttaacctgtttgacaaagagctgaacaagaaagaaattaaagatctgtacgacaaccagagcaatagcggtattctgaaagatttctggggtgattatctgcagtatgacaaaccgtattatatgctgaatctgtatgacccgaataagtatctggatgtgaataatgttggcatccgtggctatatgtatctgaaaggtccgcgtggtcgtattgtgaccaccaacatttatctgaatagcaccctgtatatgggcaccaaattcatcattaagaaatatgccagcggcaacaaagataacattgtgcgtaataatgatcgcgtgtatattaacgtggtggtgaagaataaagaatatcgcctggcaaccaatgcaagccaggcaggcgttgaaaaaattctgagcgcagttgaaatcccggatgttggtaatctgagccaggttgttgtgatgaaaagcgaaaatgatcagggcattcgcaacaagtgtaaaatgaatctgcaagacaataacggcaacgatattggctttatcggctttcaccagtttaataacattgcaaaactggtggccagcaactggtataaccgtcagattggtaaagcaagccgtacctttggttgtagctgggaatttatcccggttgatgatggttggggtgaaagcagcctggaaaatctgtatttccagggtgccagtcatcatcaccaccatcaccatcactga

SEQ ID NO: 26 - protein, 1305 aa, Artificial Sequence
  Polypeptide Sequence of rBoNT/FA(0) (His-tagged)
MPVVINSFNYDDPVNDNTIIYIRPPYYETSNTYFKAFQIMDNVWIIPERYRLGIDPSLFNPPVSLKAGSDGYFDPNYLSTNTEKNKYLQIMIKLFKRINSKPAGQILLEEIKNAIPYLGNSYTQEEQFTTNNRTVSFNVKLANGNIVQQMANLIIWGPGPDLTTNKTGGIIYSPYQSMEATPYKDGFGSIMTVEFSPEYATAFNDISIASHSPSLFIKDPALILMHQLIYVLHGLYGTYITEYKITPNVVQSYMKVTKPITSAEFLTFGGRDRNIVPQSIQSQLYNKVLSDYKRIASRLNKVNTATALINIDEFKNLYEWKYQFAKDSNGVYSVDLNKFEQLYKKIYSFTEFNLAYEFKIKTRLGYLAENFGPFYLPNLLDDSIYTEVDGFNIGALSINYQGQNIGSDINSIKKLQGQGVVSRVVRLCSNSNTKNSLCITVNNRDLFFIASQESYGENTINTYKEIDDTTTLDPSFEDILDKVILNFNEQVIPQMPNRNVSTDIQKDNYIPKYDYNRTDIIDSYEVGRNYNTFFYLNAQKFSPNESNITLTSSFDTGLLEGSKVYTFFSSDFINNINKPVQALLFIEWVKQVIRDFTTEATKTSTVDKLKDISLVVPYIGLALNIGDEIYKQHFAEAVELVGAGLLLEFSPEFLIPTLLIFTIKGYLTGSIRDKDKIIKTLDNALNVRDQKWKELYRWVVSKWLTTINTQFNKRKEQMYKALKNQATAIKKIIENKYNNYTTDEKSKIDSSYNINEIERTLNEKINLAMKNIEQFITESSIAYLINIINNETIQKLKSYDDLVRRYLLGYIRNHSSILGNSVEELNSKVNNHLDNGIPFELSSYTNDSLLIRYFNKNYGELKYNCILNIKYEMDRDKLVDSSGYRSRINIGTGVKFSEIDKNQVQLSNLESSKIEVILNNGVIYNSMYENFSTSFWIRIPKYFRNINNEYKIISCMQNNSGWEVSLNFSNMNSKIIWTLQDTEGIKKTVVFQYTQNINISDYINRWIFVTITNNRLSNSKIYINGRLINEESISDLGNIHASNNIMFKLDGCRDPHRYIWIKYFNLFDKELNKKEIKDLYDNQSNSGILKDFWGDYLQYDKPYYMLNLYDPNKYLDVNNVGIRGYMYLKGPRGRIVTTNIYLNSTLYMGTKFIIKKYASGNKDNIVRNNDRVYINVVVKNKEYRLATNASQAGVEKILSAVEIPDVGNLSQVVVMKSENDQGIRNKCKMNLQDNNGNDIGFIGFHQFNNIAKLVASNWYNRQIGKASRTFGCSWEFIPVDDGWGESSLENLYFQGASHHHHHHHH

SEQ ID NO: 27 - DNA, 2634 bp, Artificial Sequence
  Nucleotide Sequence of rLHN/FA (His-tagged)
atgccggttgtgattaacagcttcaattatgatgatccggtgaacgataacaccatcatttatatccgtccgccttattatgaaaccagcaacacctatttcaaagccttccagattatggataacgtgtggattattccggaacgttatcgtctgggtattgatccgagcctgtttaatccgcctgttagcctgaaagcaggtagtgatggttattttgatccgaattatctgagcaccaacaccgagaaaaacaaatacctgcagattatgatcaagctgttcaaacgcattaatagcaaaccggcaggtcagattctgctggaagaaatcaaaaatgcaattccgtatctgggcaacagctatacccaagaagaacagtttaccaccaataatcgtaccgtgagctttaatgttaaactggccaatggtaatatcgttcagcagatggcaaatctgattatttggggtccgggtcctgatctgaccacaaataaaaccggtggtatcatctatagcccgtatcagagcatggaagcaaccccgtataaagatggttttggtagcattatgaccgtggaatttagtccggaatatgcaaccgcctttaacgatatttcaattgcaagccatagtccgtcgctgtttatcaaagatccggcactgattctgatgcatgaactgattcatgttctgcatggtctgtatggcacctatattaccgaatacaaaattaccccgaatgtggtgcagagctatatgaaagttaccaaaccgattaccagcgcagaatttctgacctttggtggtcgtgatcgcaatattgttccgcagagcattcagagccagctgtataacaaagttctgagcgattataaacgtattgccagccgtctgaataaagttaataccgcaaccgcactgatcaacatcgatgaattcaaaaacctgtacgagtggaaataccagtttgccaaagatagcaatggtgtgtatagcgtggatctgaacaaatttgagcagctgtacaaaaaaatctatagcttcaccgaattcaacctggcctatgagtttaaaatcaaaacccgtctgggttatctggccgaaaattttggtccgttttatctgccgaatctgctggatgatagcatttataccgaagtggatggttttaacattggtgcactgagcattaactatcagggtcagaatattggcagcgatatcaacagcatcaaaaaactgcaaggtcagggtgttgttagccgtgttgttcgtctgtgtagcaatagcaataccaaaaacagcctgtgcattaccgttaataatcgcgacctgttttttatcgcaagccaagaaagctatggcgagaataccattaacacctataaagagattgacgataccaccacactggatccgagctttgaagatattctggataaagtgatcctgaacttcaacgaacaggttattccgcagatgccgaatcgtaatgttagcaccgatattcagaaagacaactacatcccgaaatacgattataaccgcaccgacattatcgatagctatgaagttggtcgcaactacaacacctttttctatctgaatgcccagaaatttagcccgaacgaaagcaatattaccctgaccagcagctttgatacaggtctgttagaaggtagcaaagtgtatacctttttcagcagcgatttcattaacaacatcaacaaaccggttcaggccctgctgtttattgaatgggttaaacaggtgattcgcgattttaccaccgaagcaaccaaaacctcaaccgttgataaactgaaagatattagcctggtggtgccgtatattggtctggcactgaatattggtgatgagatctacaaacagcattttgcagaagcagttgaactggttggtgcaggtctgctgctggaattttcaccggaatttcttattccgacgctgctgatttttaccatcaaaggttatctgaccggtagcattcgcgataaagacaaaatcattaaaaccctggataacgccctgaatgttcgtgatcagaaatggaaagaactgtatcgttgggttgttagcaaatggctgaccaccattaatacgcagttcaacaaacgcaaagaacaaatgtacaaagccctgaaaaatcaggccaccgccattaaaaagatcatcgagaacaaatataacaactataccaccgatgaaaaaagcaagatcgatagcagctataacatcaacgaaattgaacgcaccctgaacgaaaaaatcaatctggccatgaaaaacatcgagcagtttattacagaaagcagcattgcctacctgatcaatatcatcaacaacgaaaccattcagaaactgaaaagctatgatgacctggttcgtcgttatctgctgggttatattcgtaatcatagcagcattctgggcaatagcgttgaagaactgaattccaaagtgaacaaccatctggataatggcattccgtttgaactgagcagttataccaatgatagcctgctgatccgctacttcaataaaaactatggcgaagagaacctgtatttccagggtgccagtcatcatcaccaccatcaccatcactga

SEQ ID NO: 28 - protein, 877 aa, Artificial Sequence
  Polypeptide Sequence of rLHN/FA (His-tagged)
MPVVINSFNYDDPVNDNTIIYIRPPYYETSNTYFKAFQIMDNVWIIPERYRLGIDPSLFNPPVSLKAGSDGYFDPNYLSTNTEKNKYLQIMIKLFKRINSKPAGQILLEEIKNAIPYLGNSYTQEEQFTTNNRTVSFNVKLANGNIVQQMANLIIWGPGPDLTTNKTGGIIYSPYQSMEATPYKDGFGSIMTVEFSPEYATAFNDISIASHSPSLFIKDPALILMHELIHVLHGLYGTYITEYKITPNVVQSYMKVTKPITSAEFLTFGGRDRNIVPQSIQSQLYNKVLSDYKRIASRLNKVNTATALINIDEFKNLYEWKYQFAKDSNGVYSVDLNKFEQLYKKIYSFTEFNLAYEFKIKTRLGYLAENFGPFYLPNLLDDSIYTEVDGFNIGALSINYQGQNIGSDINSIKKLQGQGVVSRVVRLCSNSNTKNSLCITVNNRDLFFIASQESYGENTINTYKEIDDTTTLDPSFEDILDKVILNFNEQVIPQMPNRNVSTDIQKDNYIPKYDYNRTDIIDSYEVGRNYNTFFYLNAQKFSPNESNITLTSSFDTGLLEGSKVYTFFSSDFINNINKPVQALLFIEWVKQVIRDFTTEATKTSTVDKLKDISLVVPYIGLALNIGDEIYKQHFAEAVELVGAGLLLEFSPEFLIPTLLIFTIKGYLTGSIRDKDKIIKTLDNALNVRDQKWKELYRWVVSKWLTTINTQFNKRKEQMYKALKNQATAIKKIIENKYNNYTTDEKSKIDSSYNINEIERTLNEKINLAMKNIEQFITESSIAYLINIINNETIQKLKSYDDLVRRYLLGYIRNHSSILGNSVEELNSKVNNHLDNGIPFELSSYTNDSLLIRYFNKNYGEENLYFQGASHHHHHHHH

SEQ ID NO: 29 - DNA, 1341 bp, Artificial Sequence
  Nucleotide Sequence of rHC/FA (His-tagged)
atgctgaagtataactgcatcctgaacatcaaatatgagatggatcgtgataaactggttgatagcagcggttatcgtagccgtatcaatattggcaccggtgtgaaatttagcgagatcgataaaaatcaggtgcagctgagcaatctggaaagcagcaaaattgaagtgattctgaataacggcgtgatctacaatagcatgtatgaaaacttttcgaccagcttctggattcgcattccgaaatactttcgcaacatcaacaacgagtacaagattatcagctgtatgcagaataatagcggttgggaagttagcctgaatttcagcaatatgaacagcaaaatcatttggaccctgcaggataccgaaggtatcaaaaaaaccgttgtgtttcagtacacccagaacattaacatcagcgattacattaaccgctggatctttgtgaccattaccaataatcgtctgagcaacagcaagatctatattaacggtcgcctgattaacgaagagagcattagcgatctgggtaatattcatgccagcaacaacatcatgtttaaactggatggttgtcgtgatccgcatcgttatatttggatcaaatacttcaacctgtttgataaagaactgaacaaaaaagaaatcaaagacctgtatgataaccagagcaatagcggcattctgaaagatttttggggtgattatctgcagtatgacaaaccgtattacatgctgaatctgtacgatccgaacaaatatctggatgtgaataatgtgggtatccgtggctatatgtatctgaaaggtccgcgtggtcgtattgttaccaccaacatttatctgaatagcaccctgtatatgggcaccaaattcatcattaaaaagtatgccagcggcaacaaagataacattgtgcgtaataatgatcgcgtgtatatcaatgtggtggtgaagaataaagaatatcgtctggccaccaatgcaagccaggcaggcgttgaaaaaattctgagcgcagttgaaattccggatgttggtaatctgagccaggttgttgttatgaaaagcgaaaatgatcagggcattcgcaacaaatgcaaaatgaatctgcaggacaataacggcaacgatattggttttattggcttccaccagttcaacaacattgcaaaactggtggcgagcaattggtataatcgtcagattggtaaagcaagccgtacctttggttgtagctgggaatttattccggttgatgatggttggggtgaaagcagcctggaaaatctgtattttcagggtgcaagtcatcatcaccaccatcaccatcattaa

SEQ ID NO: 30 - protein, 446 aa, Artificial Sequence
  Polypeptide Sequence of rHC/FA (His-tagged)
MLKYNCILNIKYEMDRDKLVDSSGYRSRINIGTGVKFSEIDKNQVQLSNLESSKIEVILNNGVIYNSMYENFSTSFWIRIPKYFRNINNEYKIISCMQNNSGWEVSLNFSNMNSKIIWTLQDTEGIKKTVVFQYTQNINISDYINRWIFVTITNNRLSNSKIYINGRLINEESISDLGNIHASNNIMFKLDGCRDPHRYIWIKYFNLFDKELNKKEIKDLYDNQSNSGILKDFWGDYLQYDKPYYMLNLYDPNKYLDVNNVGIRGYMYLKGPRGRIVTTNIYLNSTLYMGTKFIIKKYASGNKDNIVRNNDRVYINVVVKNKEYRLATNASQAGVEKILSAVEIPDVGNLSQVVVMKSENDQGIRNKCKMNLQDNNGNDIGFIGFHQFNNIAKLVASNWYNRQIGKASRTFGCSWEFIPVDDGWGESSLENLYFQGASHHHHHHHH

SEQ ID NO: 31 - DNA, 1347 bp, Artificial Sequence
  Nucleotide Sequence of rLC/FA (His-tagged)
atgccggttgtgattaacagcttcaattatgatgatccggtgaacgataacaccatcatttatatccgtccgccttattatgaaaccagcaacacctatttcaaagccttccagattatggataacgtgtggattattccggaacgttatcgtctgggtattgatccgagcctgtttaatccgcctgttagcctgaaagcaggtagtgatggttattttgatccgaattatctgagcaccaacaccgagaaaaacaaatacctgcagattatgatcaagctgttcaaacgcattaatagcaaaccggcaggtcagattctgctggaagaaatcaaaaatgcaattccgtatctgggcaacagctatacccaagaagaacagtttaccaccaataatcgtaccgtgagctttaatgttaaactggccaatggtaatatcgttcagcagatggcaaatctgattatttggggtccgggtcctgatctgaccacaaataaaaccggtggtatcatctatagcccgtatcagagcatggaagcaaccccgtataaagatggttttggtagcattatgaccgtggaatttagtccggaatatgcaaccgcctttaacgatatttcaattgcaagccatagtccgtcgctgtttatcaaagatccggcactgattctgatgcatgaactgattcatgttctgcatggtctgtatggcacctatattaccgaatacaaaattaccccgaatgtggtgcagagctatatgaaagttaccaaaccgattaccagcgcagaatttctgacctttggtggtcgtgatcgcaatattgttccgcagagcattcagagccagctgtataacaaagttctgagcgattataaacgtattgccagccgtctgaataaagttaataccgcaaccgcactgatcaacatcgatgaattcaaaaacctgtacgagtggaaataccagtttgccaaagatagcaatggtgtgtatagcgtggatctgaacaaatttgagcagctgtacaaaaaaatctatagcttcaccgaattcaacctggcctatgagtttaaaatcaaaacccgtctgggttatctggccgaaaattttggtccgttttatctgccgaatctgctggatgatagcatttataccgaagtggatggttttaacattggtgcactgagcattaactatcagggtcagaatattggcagcgatatcaacagcatcaaaaaactgcaaggtcagggtgttgttagccgtgttgttcgtctgtgtagcaatagcgaaaatctgtattttcagggtgccagtcatcatcaccaccatcaccatcactga

SEQ ID NO: 32 - protein, 448 aa, Artificial Sequence
  Polypeptide Sequence of rLC/FA (His-tagged)
MPVVINSFNYDDPVNDNTIIYIRPPYYETSNTYFKAFQIMDNVWIIPERYRLGIDPSLFNPPVSLKAGSDGYFDPNYLSTNTEKNKYLQIMIKLFKRINSKPAGQILLEEIKNAIPYLGNSYTQEEQFTTNNRTVSFNVKLANGNIVQQMANLIIWGPGPDLTTNKTGGIIYSPYQSMEATPYKDGFGSIMTVEFSPEYATAFNDISIASHSPSLFIKDPALILMHELIHVLHGLYGTYITEYKITPNVVQSYMKVTKPITSAEFLTFGGRDRNIVPQSIQSQLYNKVLSDYKRIASRLNKVNTATALINIDEFKNLYEWKYQFAKDSNGVYSVDLNKFEQLYKKIYSFTEFNLAYEFKIKTRLGYLAENFGPFYLPNLLDDSIYTEVDGFNIGALSINYQGQNIGSDINSIKKLQGQGVVSRVVRLCSNSENLYFQGASHHHHHHHH

SEQ ID NO: 33 - DNA, 3888 bp, Artificial Sequence
  Nucleotide Sequence of rBoNT/F(0) (His-tagged)
atgccggttgtgattaacagcttcaattataacgatccggtgaacgatgataccatcctgtatatgcagattccgtatgaagagaaaagcaaaaagtactacaaagcctttgagatcatgcgcaacgtttggattattccggaacgtaataccattggcaccgatccgagcgattttgatccgcctgcaagcctggaaaatggtagcagcgcatattatgatccgaattatctgaccaccgatgccgaaaaagatcgttatctgaaaaccaccatcaaactgttcaaacgcattaatagcaatccggcaggcgaagttctgctgcaagaaattagctatgcaaaaccgtatctgggcaatgaacataccccgattaatgaatttcatccggttacacgtaccacgagcgttaacattaaaagcagcaccaatgtgaagtccagcattattctgaatctgctggttttaggtgcaggtccggatatttttgaaaattcaagctatccggtgcgcaaactgatggatagcggtggtgtgtatgatccgtcaaatgatggttttggcagcattaacattgtgacctttagtccggaatatgaatacaccttcaacgatattagcggtggctataatagcagcaccgaaagttttattgcagatccggcaattagcctggcacaccagctgatttatgcactgcatggtctgtatggtgcacgtggtgttacctataaagaaaccattaaagttaaacaggcaccgctgatgattgcggaaaaaccgattcgtctggaagaatttctgacctttggtggtcaggatctgaacattattaccagcgcaatgaaagagaaaatctataataacctgctggccaactatgagaaaattgcaacccgtctgagccgtgttaatagcgcacctcctgaatatgatatcaacgagtataaagactattttcagtggaaatacggcctggataaaaatgcagatggtagctataccgtgaacgagaacaaatttaacgagatctacaaaaaactgtatagcttcaccgaaatcgatctggccaacaaattcaaagtgaaatgccgcaacacctacttcatcaaatatggctttctgaaagttccgaacctgcttgatgatgatatctataccgttagcgaaggctttaacattggtaatctggccgttaataatcgcggtcagaacattaaactgaacccgaaaattatcgatagcatcccggataaaggcctggttgaaaaaattgtgaaattctgcaaaagcgtgattccgcgtaaaggcaccaaagcaccgcctcgtctgtgtattcgtgtgaataatcgtgaactgttttttgttgcaagcgagagcagctataacgagaatgatattaacaccccgaaagagattgacgataccaccaatctgaataacaactatcgcaacaatctggatgaagtgatcctggattataacagcgaaaccattccgcagattagcaatcagaccctgaataccctggttcaggatgatagctatgttccgcgttatgatagcaatggcaccagcgaaattgaagaacataatgtggttgatctgaacgtgttcttttatctgcatgcacagaaagtgccggaaggtgaaaccaatattagcctgaccagcagcattgataccgcactgagcgaagaaagccaggtttataccttttttagcagcgaattcatcaacaccattaacaaaccggttcatgcagcactgtttattagctggattaatcaggtgattcgcgattttaccaccgaagcaacccagaaaagcacctttgataaaattgccgatattagtctggtggtgccgtatgttggtctggcactgaatattggtaatgaagtgcagaaagagaactttaaagaagccttcgaactgttaggtgccggtattctgctggaatttgtgccggaactgctgattccgaccattctggtttttaccattaagagctttattggcagcagcgagaacaagaacaaaatcattaaagccatcaacaacagcctgatggaacgcgaaaccaaatggaaagaaatttacagctggattgtgagcaattggctgacccgtatcaatacccagtttaacaaacgcaaagaacaaatgtatcaggccctgcagaatcaggttgatgcaattaaaaccgtgatcgaatacaaatacaacaactataccagcgacgaacgtaatcgcctggaaagcgaatacaacattaataacattcgcgaagaactgaacaaaaaagtgagcctggcaatggaaaacatcgaacgttttattaccgaaagcagcatcttctacctgatgaaactgattaacgaagccaaagttagcaaactgcgcgaatatgatgaaggcgttaaagaatatctgctggactatattagcgaacatcgtagcattctgggtaatagcgttcaagagctgaatgatctggttaccagcacactgaataatagcattccgtttgaactgagcagctacaccaacgataaaatcctgatcctgtacttcaacaaactgtacaagaagatcaaggacaacagcatactggatatgcgctatgaaaacaacaagttcattgatatcagcggctatggtagcaacattagcattaatggtgatgtgtatatctacagcaccaaccgcaatcagtttggtatttatagcagcaaaccgagcgaagttaatattgcgcagaataacgatatcatctacaacggtcgctatcagaactttagcattagcttttgggttcgcattccgaaatactttaacaaggtgaacctgaacaacgagtacaccattattgattgcattcgcaataataacagcggctggaaaatcagcctgaactataacaaaattatctggaccctgcaggataccgcaggtaataatcagaaactggtgtttaactacacccagatgattagcatcagcgactatatcaacaaatggatctttgtgaccattaccaacaatcgtctgggtaacagccgcatttatatcaatggcaatctgatcgacgaaaaaagcatttcaaatctgggcgatattcacgtgagcgataacattctgttcaaaattgttggctgcaacgatacccgttatgttggtattcgttacttcaaagtgtttgatacggaactgggcaaaacggaaattgaaaccctgtatagtgatgaaccggatccgagcattctgaaagatttttggggtaattatctgctgtacaacaaacgctactatctgctgaacctgctgcgtaccgataaaagcattacacagaatagcaactttctgaacatcaatcagcagcgtggtgtttatcagaaaccgaacatttttagcaacacccgtctgtataccggtgtggaagttattattcgtaaaaacggtagcaccgatatcagcaacaccgataactttgtgcgtaaaaatgacctggcctatattaacgttgttgatcgtgatgttgagtatcgtctgtatgcggatattagcattgccaaaccggaaaagattatcaaactgatccgtaccagcaacagcaataattcactgggtcagattatcgtgatggacagcattggtaacaattgcaccatgaatttccagaacaataacggtggtaatattggcctgctgggctttcatagcaataatctggttgcaagcagctggtattacaacaacatccgtaaaaataccagcagtaatggttgcttttggagctttatcagtaaagaacatggctggcaagaaaacgagaacctgtattttcagggtgcaagtcatcatcaccatcaccaccatcattaa

SEQ ID NO: 34 - protein, 1295 aa, Artificial Sequence
  Polypeptide Sequence of rBoNT/F(0) (His-tagged)
MPVVINSFNYNDPVNDDTILYMQIPYEEKSKKYYKAFEIMRNVWIIPERNTIGTDPSDFDPPASLENGSSAYYDPNYLTTDAEKDRYLKTTIKLFKRINSNPAGEVLLQEISYAKPYLGNEHTPINEFHPVTRTTSVNIKSSTNVKSSIILNLLVLGAGPDIFENSSYPVRKLMDSGGVYDPSNDGFGSINIVTFSPEYEYTFNDISGGYNSSTESFIADPAISLAHQLIYALHGLYGARGVTYKETIKVKQAPLMIAEKPIRLEEFLTFGGQDLNIITSAMKEKIYNNLLANYEKIATRLSRVNSAPPEYDINEYKDYFQWKYGLDKNADGSYTVNENKFNEIYKKLYSFTEIDLANKFKVKCRNTYFIKYGFLKVPNLLDDDIYTVSEGFNIGNLAVNNRGQNIKLNPKIIDSIPDKGLVEKIVKFCKSVIPRKGTKAPPRLCIRVNNRELFFVASESSYNENDINTPKEIDDTTNLNNNYRNNLDEVILDYNSETIPQISNQTLNTLVQDDSYVPRYDSNGTSEIEEHNVVDLNVFFYLHAQKVPEGETNISLTSSIDTALSEESQVYTFFSSEFINTINKPVHAALFISWINQVIRDFTTEATQKSTFDKIADISLVVPYVGLALNIGNEVQKENFKEAFELLGAGILLEFVPELLIPTILVFTIKSFIGSSENKNKIIKAINNSLMERETKWKEIYSWIVSNWLTRINTQFNKRKEQMYQALQNQVDAIKTVIEYKYNNYTSDERNRLESEYNINNIREELNKKVSLAMENIERFITESSIFYLMKLINEAKVSKLREYDEGVKEYLLDYISEHRSILGNSVQELNDLVTSTLNNSIPFELSSYTNDKILILYFNKLYKKIKDNSILDMRYENNKFIDISGYGSNISINGDVYIYSTNRNQFGIYSSKPSEVNIAQNNDIIYNGRYQNFSISFWVRIPKYFNKVNLNNEYTIIDCIRNNNSGWKISLNYNKIIWTLQDTAGNNQKLVFNYTQMISISDYINKWIFVTITNNRLGNSRIYINGNLIDEKSISNLGDIHVSDNILFKIVGCNDTRYVGIRYFKVFDTELGKTEIETLYSDEPDPSILKDFWGNYLLYNKRYYLLNLLRTDKSITQNSNFLNINQQRGVYQKPNIFSNTRLYTGVEVIIRKNGSTDISNTDNFVRKNDLAYINVVDRDVEYRLYADISIAKPEKIIKLIRTSNSNNSLGQIIVMDSIGNNCTMNFQNNNGGNIGLLGFHSNNLVASSWYYNNIRKNTSSNGCFWSFISKEHGWQENENLYFQGASHHHHHHHH

SEQ ID NO: 35 - DNA, 2649 bp, Artificial Sequence
  Nucleotide Sequence of rLHN/F (His-tagged)
atgccggttgtgattaacagcttcaattataacgatccggtgaacgatgataccatcctgtatatgcagattccgtatgaagagaaaagcaaaaagtactacaaagcctttgagatcatgcgcaacgtttggattattccggaacgtaataccattggcaccgatccgagcgattttgatccgcctgcaagcctggaaaatggtagcagcgcatattatgatccgaattatctgaccaccgatgccgaaaaagatcgttatctgaaaaccaccatcaaactgttcaaacgcattaatagcaatccggcaggcgaagttctgctgcaagaaattagctatgcaaaaccgtatctgggcaatgaacataccccgattaatgaatttcatccggttacacgtaccacgagcgttaacattaaaagcagcaccaatgtgaagtccagcattattctgaatctgctggttttaggtgcaggtccggatatttttgaaaattcaagctatccggtgcgcaaactgatggatagcggtggtgtgtatgatccgtcaaatgatggttttggcagcattaacattgtgacctttagtccggaatatgaatacaccttcaacgatattagcggtggctataatagcagcaccgaaagttttattgcagatccggcaattagcctggcacatgaactgattcatgcactgcatggtctgtatggtgcacgtggtgttacctataaagaaaccattaaagttaaacaggcaccgctgatgattgcggaaaaaccgattcgtctggaagaatttctgacctttggtggtcaggatctgaacattattaccagcgcaatgaaagagaaaatctataataacctgctggccaactatgagaaaattgcaacccgtctgagccgtgttaatagcgcacctcctgaatatgatatcaacgagtataaagactattttcagtggaaatacggcctggataaaaatgcagatggtagctataccgtgaacgagaacaaatttaacgagatctacaaaaaactgtatagcttcaccgaaatcgatctggccaacaaattcaaagtgaaatgccgcaacacctacttcatcaaatatggctttctgaaagttccgaacctgcttgatgatgatatctataccgttagcgaaggctttaacattggtaatctggccgttaataatcgcggtcagaacattaaactgaacccgaaaattatcgatagcatcccggataaaggcctggttgaaaaaattgtgaaattctgcaaaagcgtgattccgcgtaaaggcaccaaagcaccgcctcgtctgtgtattcgtgtgaataatcgtgaactgttttttgttgcaagcgagagcagctataacgagaatgatattaacaccccgaaagagattgacgataccaccaatctgaataacaactatcgcaacaatctggatgaagtgatcctggattataacagcgaaaccattccgcagattagcaatcagaccctgaataccctggttcaggatgatagctatgttccgcgttatgatagcaatggcaccagcgaaattgaagaacataatgtggttgatctgaacgtgttcttttatctgcatgcacagaaagtgccggaaggtgaaaccaatattagcctgaccagcagcattgataccgcactgagcgaagaaagccaggtttataccttttttagcagcgaattcatcaacaccattaacaaaccggttcatgcagcactgtttattagctggattaatcaggtgattcgcgattttaccaccgaagcaacccagaaaagcacctttgataaaattgccgatattagtctggtggtgccgtatgttggtctggcactgaatattggtaatgaagtgcagaaagagaactttaaagaagccttcgaactgttaggtgccggtattctgctggaatttgtgccggaactgctgattccgaccattctggtttttaccattaagagctttattggcagcagcgagaacaagaacaaaatcattaaagccatcaacaacagcctgatggaacgcgaaaccaaatggaaagaaatttacagctggattgtgagcaattggctgacccgtatcaatacccagtttaacaaacgcaaagaacaaatgtatcaggccctgcagaatcaggttgatgcaattaaaaccgtgatcgaatacaaatacaacaactataccagcgacgaacgtaatcgcctggaaagcgaatacaacattaataacattcgcgaagaactgaacaaaaaagtgagcctggcaatggaaaacatcgaacgttttattaccgaaagcagcatcttctacctgatgaaactgattaacgaagccaaagttagcaaactgcgcgaatatgatgaaggcgttaaagaatatctgctggactatattagcgaacatcgtagcattctgggtaatagcgttcaagagctgaatgatctggttaccagcacactgaataatagcattccgtttgaactgagcagctacaccaacgataaaatcctgatcctgtacttcaacaaactgtacaagaaagaaaacctgtattttcagggtgcaagccatcatcaccaccatcaccatcattaa

SEQ ID NO: 36 - protein, 882 aa, Artificial Sequence
  Polypeptide Sequence of rLHN/F (His-tagged)
MPVVINSFNYNDPVNDDTILYMQIPYEEKSKKYYKAFEIMRNVWIIPERNTIGTDPSDFDPPASLENGSSAYYDPNYLTTDAEKDRYLKTTIKLFKRINSNPAGEVLLQEISYAKPYLGNEHTPINEFHPVTRTTSVNIKSSTNVKSSIILNLLVLGAGPDIFENSSYPVRKLMDSGGVYDPSNDGFGSINIVTFSPEYEYTFNDISGGYNSSTESFIADPAISLAHELIHALHGLYGARGVTYKETIKVKQAPLMIAEKPIRLEEFLTFGGQDLNIITSAMKEKIYNNLLANYEKIATRLSRVNSAPPEYDINEYKDYFQWKYGLDKNADGSYTVNENKFNEIYKKLYSFTEIDLANKFKVKCRNTYFIKYGFLKVPNLLDDDIYTVSEGFNIGNLAVNNRGQNIKLNPKIIDSIPDKGLVEKIVKFCKSVIPRKGTKAPPRLCIRVNNRELFFVASESSYNENDINTPKEIDDTTNLNNNYRNNLDEVILDYNSETIPQISNQTLNTLVQDDSYVPRYDSNGTSEIEEHNVVDLNVFFYLHAQKVPEGETNISLTSSIDTALSEESQVYTFFSSEFINTINKPVHAALFISWINQVIRDFTTEATQKSTFDKIADISLVVPYVGLALNIGNEVQKENFKEAFELLGAGILLEFVPELLIPTILVFTIKSFIGSSENKNKIIKAINNSLMERETKWKEIYSWIVSNWLTRINTQFNKRKEQMYQALQNQVDAIKTVIEYKYNNYTSDERNRLESEYNINNIREELNKKVSLAMENIERFITESSIFYLMKLINEAKVSKLREYDEGVKEYLLDYISEHRSILGNSVQELNDLVTSTLNNSIPFELSSYTNDKILILYFNKLYKKENLYFQGASHHHHHHHH

SEQ ID NO: 37 - DNA, 1296 bp, Artificial Sequence
  Nucleotide Sequence of rHC/F (His-tagged)
atgatcaaggataacagcattctggatatgcgctatgagaacaacaaattcattgatattagcggctatggcagcaacattagcattaatggtgatgtgtatatctacagcaccaaccgtaatcagtttggcatttatagcagcaaaccgagcgaagttaatattgcccagaacaacgatatcatctataacggtcgctatcagaacttcagcattagcttttgggttcgcattccgaaatacttcaataaggtgaacctgaacaacgagtataccatcattgattgcattcgcaataataacagcggctggaaaattagcctgaactacaacaaaattatctggaccctgcaggataccgcaggtaataatcagaaactggtgtttaactacacccagatgattagcatcagcgactatatcaacaaatggatctttgtgaccattaccaataatcgcctgggtaatagccgcatttatatcaatggtaacctgatcgatgagaaaagcattagcaatctgggtgatattcatgtgagcgataacatcctgtttaaaatcgtgggttgtaacgatacccgttatgttggtattcgctacttcaaagtgtttgataccgaactgggtaaaaccgaaattgaaaccctgtatagtgatgaaccggatccgagcattctgaaagatttttggggtaattatctgctgtacaacaaacgctactatctgctgaatctgctgcgtaccgataaatcaattacccagaatagcaacttcctgaacattaatcagcagcgtggtgtttatcagaaaccgaacatttttagcaacacccgtctgtataccggtgtggaagttattattcgtaaaaatggcagcaccgatatcagcaacaccgataactttgttcgcaaaaatgatctggcgtatatcaacgttgttgatcgtgatgttgaatatcgtctgtatgccgatattagcattgccaaaccggaaaaaatcatcaaactgatccgtaccagcaacagcaataattcactgggtcagattattgtgatggatagcattggtaataactgcaccatgaactttcagaacaataacggtggtaatattggtctgctgggctttcatagtaataatctggttgcaagcagctggtattataacaacatccgtaaaaataccagcagcaatggttgcttttggagctttattagcaaagaacatggctggcaagaaaacgagaatctgtattttcagggtgcaagtcatcatcaccaccatcaccatcattaa

SEQ ID NO: 38 - protein, 431 aa, Artificial Sequence
  Polypeptide Sequence of rHC/F (His-tagged)
MIKDNSILDMRYENNKFIDISGYGSNISINGDVYIYSTNRNQFGIYSSKPSEVNIAQNNDIIYNGRYQNFSISFWVRIPKYFNKVNLNNEYTIIDCIRNNNSGWKISLNYNKIIWTLQDTAGNNQKLVFNYTQMISISDYINKWIFVTITNNRLGNSRIYINGNLIDEKSISNLGDIHVSDNILFKIVGCNDTRYVGIRYFKVFDTELGKTEIETLYSDEPDPSILKDFWGNYLLYNKRYYLLNLLRTDKSITQNSNFLNINQQRGVYQKPNIFSNTRLYTGVEVIIRKNGSTDISNTDNFVRKNDLAYINVVDRDVEYRLYADISIAKPEKIIKLIRTSNSNNSLGQIIVMDSIGNNCTMNFQNNNGGNIGLLGFHSNNLVASSWYYNNIRKNTSSNGCFWSFISKEHGWQENENLYFQGASHHHHHHHH

SEQ ID NO: 39 - DNA, 1347 bp, Artificial Sequence
  Nucleotide Sequence of rLC/F (His-tagged)
atgccggttgtgattaacagcttcaattataacgatccggtgaacgatgataccatcctgtatatgcagattccgtatgaagagaaaagcaaaaagtactacaaagcctttgagatcatgcgcaacgtttggattattccggaacgtaataccattggcaccgatccgagcgattttgatccgcctgcaagcctggaaaatggtagcagcgcatattatgatccgaattatctgaccaccgatgccgaaaaagatcgttatctgaaaaccaccatcaaactgttcaaacgcattaatagcaatccggcaggcgaagttctgctgcaagaaattagctatgcaaaaccgtatctgggcaatgaacataccccgattaatgaatttcatccggttacacgtaccacgagcgttaacattaaaagcagcaccaatgtgaagtccagcattattctgaatctgctggttttaggtgcaggtccggatatttttgaaaattcaagctatccggtgcgcaaactgatggatagcggtggtgtgtatgatccgtcaaatgatggttttggcagcattaacattgtgacctttagtccggaatatgaatacaccttcaacgatattagcggtggctataatagcagcaccgaaagttttattgcagatccggcaattagcctggcacatgaactgattcatgcactgcatggtctgtatggtgcacgtggtgttacctataaagaaaccattaaagttaaacaggcaccgctgatgattgcggaaaaaccgattcgtctggaagaatttctgacctttggtggtcaggatctgaacattattaccagcgcaatgaaagagaaaatctataataacctgctggccaactatgagaaaattgcaacccgtctgagccgtgttaatagcgcacctcctgaatatgatatcaacgagtataaagactattttcagtggaaatacggcctggataaaaatgcagatggtagctataccgtgaacgagaacaaatttaacgagatctacaaaaaactgtatagcttcaccgaaatcgatctggccaacaaattcaaagtgaaatgccgcaacacctacttcatcaaatatggctttctgaaagttccgaacctgcttgatgatgatatctataccgttagcgaaggctttaacattggtaatctggccgttaataatcgcggtcagaacattaaactgaacccgaaaattatcgatagcatcccggataaaggcctggttgaaaaaattgtgaaattctgcaaaagcgagaacctgtattttcagggtgcaagtcatcatcaccatcaccaccatcattaa

SEQ ID NO: 40 - protein, 448 aa, Artificial Sequence
  Polypeptide Sequence of rLC/F (His-tagged)
MPVVINSFNYNDPVNDDTILYMQIPYEEKSKKYYKAFEIMRNVWIIPERNTIGTDPSDFDPPASLENGSSAYYDPNYLTTDAEKDRYLKTTIKLFKRINSNPAGEVLLQEISYAKPYLGNEHTPINEFHPVTRTTSVNIKSSTNVKSSIILNLLVLGAGPDIFENSSYPVRKLMDSGGVYDPSNDGFGSINIVTFSPEYEYTFNDISGGYNSSTESFIADPAISLAHELIHALHGLYGARGVTYKETIKVKQAPLMIAEKPIRLEEFLTFGGQDLNIITSAMKEKIYNNLLANYEKIATRLSRVNSAPPEYDINEYKDYFQWKYGLDKNADGSYTVNENKFNEIYKKLYSFTEIDLANKFKVKCRNTYFIKYGFLKVPNLLDDDIYTVSEGFNIGNLAVNNRGQNIKLNPKIIDSIPDKGLVEKIVKFCKSENLYFQGASHHHHHHHH

SEQ ID NO: 41 - DNA, 1317 bp, Artificial Sequence
  Nucleotide Sequence of Cationic rHC/A (His-tagged)
atgatcatcaacaccagcattctgaacctgcgttatgaaagcaaacatctgattgatctgagccgttatgccagcaaaatcaatataggcagcaaggttaacttcgacccgattgacaaaaatcagatacagctgtttaatctggaaagcagcaaaattgaggtgatcctgaaaaaagcgatcgtgtataatagcatgtacgagaatttttcgaccagcttttggattcgcatcccgaaatactttaacaagattagcctgaacaacgagtataccatcattaactgcatggaaaacaatagcggttggaaagtcagcctgaattatggcgaaattatctggaccctgcaggataccaaagaaatcaaacagcgtgtggtgttcaaatacagccagatgattaatatcagcgactatatcaaccgctggatttttgtgaccattaccaataatcggctgaacaagagcaagatctatattaacggtcgtctgattgaccagaaaccgattagtaatctgggtaatattcatgcgagcaacaaaatcatgtttaaactggatggttgccgtgatacccatcgttatatttggatcaaatacttcaacctgttcgataaagagttgaacgaaaaagaaattaaagacctgtacgataaccagagcaatagcggcatactgaaagatttttggggagattatctgcagtatgacaaaccgtattatatgctgaatctgtacgacccgaataaatacgtggatgttaataatgtgggcatccgtggttatatgtacctgaaaggtccgcgtggtagcgttatgaccacaaacatttatctgaatagcagcctgtatcgcggaaccaaattcatcattaaaaagtatgccagcggcaacaaggataatattgtgcgtaataatgatcgcgtgtacattaacgttgtggtgaagaataaagaatatcgcctggcaaccaatgcaagccaggcaggcgttgaaaaaattctgagtgccctggaaattccggatgttggtaatctgagccaggttgttgtgatgaaaagcaaaaacgataaaggcatcaccaacaaatgcaagatgaatctgcaggacaataacggcaatgatattggcttcattggctttcaccagtttaacaacattgcaaaactggttgcgagcaattggtataatcgtcagattgaacgtagcagtcgtaccctgggttgtagctgggaatttatccctgtggatgatggttggggtgaacgtccgctgaagcttgcggccgcactcgagcaccaccaccaccaccactga

SEQ ID NO: 42 - protein, 438 aa, Artificial Sequence
  Polypeptide Sequence of Cationic rHC/A (His-tagged)
MIINTSILNLRYESKHLIDLSRYASKINIGSKVNFDPIDKNQIQLFNLESSKIEVILKKAIVYNSMYENFSTSFWIRIPKYFNKISLNNEYTIINCMENNSGWKVSLNYGEIIWTLQDTKEIKQRVVFKYSQMINISDYINRWIFVTITNNRLNKSKIYINGRLIDQKPISNLGNIHASNKIMFKLDGCRDTHRYIWIKYFNLFDKELNEKEIKDLYDNQSNSGILKDFWGDYLQYDKPYYMLNLYDPNKYVDVNNVGIRGYMYLKGPRGSVMTTNIYLNSSLYRGTKFIIKKYASGNKDNIVRNNDRVYINVVVKNKEYRLATNASQAGVEKILSALEIPDVGNLSQVVVMKSKNDKGITNKCKMNLQDNNGNDIGFIGFHQFNNIAKLVASNWYNRQIERSSRTLGCSWEFIPVDDGWGERPLKLAAALEHHHHHH

SEQ ID NO: 43 - DNA, 1341 bp, Artificial Sequence
  Nucleotide Sequence of rHC/AB (His-tagged)
atgattctgaacaatattatcctgaacctgcgttacaaagacaacaatctgatcgatctgagcggctatggtgcaaaagttgaagtctacgacggtgtcgaactgaacgataaaaaccagttcaaactgacctcatcggctaactcaaaaattcgtgtgacgcagaaccaaaacatcatcttcaactcggtctttctggacttcagcgtgtctttctggattcgcatcccgaaatataaaaatgatggcatccagaactacatccataacgaatacaccatcatcaactgtatgaaaaacaacagtggttggaaaatttccatccgtggcaaccgcattatctggaccctgattgatatcaatggtaaaacgaaaagcgtgtttttcgaatacaacatccgtgaagatatctctgaatacatcaatcgctggtttttcgtgaccattacgaacaatctgaacaatgcgaaaatctatatcaacggcaaactggaaagtaataccgacatcaaagatattcgtgaagttatcgccaacggtgaaatcatcttcaaactggatggcgacatcgatcgcacccagttcatttggatgaaatacttctccatcttcaacacggaactgagtcagtccaatatcgaagaacgctacaaaatccaatcatactcggaatacctgaaagatttctggggtaacccgctgatgtacaacaaagaatactacatgttcaacgcgggcaacaaaaactcatacatcaaactgaaaaaagattcgccggtgggtgaaatcctgacccgtagcaaatacaaccagaactctaaatacatcaactatcgcgatctgtacattggcgaaaaatttattatccgtcgcaaaagcaactctcagagtattaatgatgacatcgtgcgtaaagaagactacatctatctggatttctttaatctgaaccaagaatggcgcgtttatacctacaaatacttcaaaaaagaagaaatgaaactgttcctggccccgatttacgacagcgatgaattttacaacaccatccagatcaaagaatacgatgaacagccgacgtatagttgccaactgctgttcaaaaaagacgaagaatccaccgatgaaattggcctgattggtatccaccgtttctatgaaagcggtatcgttttcgaagaatacaaagattacttctgtatctctaaatggtatctgaaagaagtcaaacgcaaaccgtacaacctgaaactgggctgcaactggcaatttatcccgaaagacgaaggctggaccgaaaagcttgcggccgcactcgagcaccaccaccaccaccactga

SEQ ID NO: 44 - protein, 446 aa, Artificial Sequence
  Polypeptide Sequence of rHC/AB (His-tagged)
MILNNIILNLRYKDNNLIDLSGYGAKVEVYDGVELNDKNQFKLTSSANSKIRVTQNQNIIFNSVFLDFSVSFWIRIPKYKNDGIQNYIHNEYTIINCMKNNSGWKISIRGNRIIWTLIDINGKTKSVFFEYNIREDISEYINRWFFVTITNNLNNAKIYINGKLESNTDIKDIREVIANGEIIFKLDGDIDRTQFIWMKYFSIFNTELSQSNIEERYKIQSYSEYLKDFWGNPLMYNKEYYMFNAGNKNSYIKLKKDSPVGEILTRSKYNQNSKYINYRDLYIGEKFIIRRKSNSQSINDDIVRKEDYIYLDFFNLNQEWRVYTYKYFKKEEMKLFLAPIYDSDEFYNTIQIKEYDEQPTYSCQLLFKKDEESTDEIGLIGIHRFYESGIVFEEYKDYFCISKWYLKEVKRKPYNLKLGCNWQFIPKDEGWTEKLAAALEHHHHHH

SEQ ID NO: 45 - DNA, 1306 bp, Artificial Sequence
  Nucleotide Sequence of rHC/A Variant Y1117V H1253K (His-tagged)
atgatcatcaatactagcattctgaacctgcgttacgagagcaatcatctgattgatctgagccgttatgcaagcaagatcaacatcggtagcaaggtcaattttgacccgatcgataagaaccagatccagctgtttaatctggaatcgagcaaaattgaggttatcctgaaaaacgccattgtctacaactccatgtacgagaatttctccaccagcttctggattcgcatcccgaaatacttcaacagcattagcctgaacaacgagtatactatcatcaactgtatggagaacaacagcggttggaaggtgtctctgaactatggtgagatcatttggaccttgcaggacacccaagagatcaagcagcgcgtcgtgttcaagtactctcaaatgatcaacatttccgattacattaatcgttggatcttcgtgaccattacgaataaccgtctgaataacagcaagatttacatcaatggtcgcttgatcgatcagaaaccgattagcaacctgggtaatatccacgcaagcaacaacattatgttcaaattggacggttgccgcgatacccatcgttatatctggatcaagtatttcaacctgtttgataaagaactgaatgagaaggagatcaaagatttgtatgacaaccaatctaacagcggcattttgaaggacttctggggcgattatctgcaatacgataagccgtactatatgctgaacctggttgatccgaacaaatatgtggatgtcaataatgtgggtattcgtggttacatgtatttgaagggtccgcgtggcagcgttatgacgaccaacatttacctgaactctagcctgtaccgtggtacgaaattcatcattaagaaatatgccagcggcaacaaagataacattgtgcgtaataacgatcgtgtctacatcaacgtggtcgtgaagaataaagagtaccgtctggcgaccaacgcttcgcaggcgggtgttgagaaaattctgagcgcgttggagatccctgatgtcggtaatctgagccaagtcgtggttatgaagagcaagaacgaccagggtatcactaacaagtgcaagatgaacctgcaagacaacaatggtaacgacatcggctttattggtttcaaacagttcaacaatattgctaaactggtagcgagcaattggtacaatcgtcagattgagcgcagcagccgtactttgggctgtagctgggagtttatcccggtcgatgatggttggggcgaacgtccgctgcaccatcaccatcaccatcaccatcaccatt

SEQ ID NO: 46 - protein, 435 aa, Artificial Sequence
  Polypeptide Sequence of rHC/A Variant Y1117V H1253K (His-tagged)
MIINTSILNLRYESNHLIDLSRYASKINIGSKVNFDPIDKNQIQLFNLESSKIEVILKNAIVYNSMYENFSTSFWIRIPKYFNSISLNNEYTIINCMENNSGWKVSLNYGEIIWTLQDTQEIKQRVVFKYSQMINISDYINRWIFVTITNNRLNNSKIYINGRLIDQKPISNLGNIHASNNIMFKLDGCRDTHRYIWIKYFNLFDKELNEKEIKDLYDNQSNSGILKDFWGDYLQYDKPYYMLNLVDPNKYVDVNNVGIRGYMYLKGPRGSVMTTNIYLNSSLYRGTKFIIKKYASGNKDNIVRNNDRVYINVVVKNKEYRLATNASQAGVEKILSALEIPDVGNLSQVVVMKSKNDQGITNKCKMNLQDNNGNDIGFIGFKQFNNIAKLVASNWYNRQIERSSRTLGCSWEFIPVDDGWGERPLHHHHHHHHHH

SEQ ID NO: 47 - DNA, 1308 bp, Artificial Sequence
  Nucleotide Sequence of rHC/A Variant Y1117V F1252Y H1253K L1278F (His-tagged)
atgatcatcaatactagcattctgaacctgcgttacgagagcaatcatctgattgatctgagccgttatgcaagcaagatcaacatcggtagcaaggtcaattttgacccgatcgataagaaccagatccagctgtttaatctggaatcgagcaaaattgaggttatcctgaaaaacgccattgtctacaactccatgtacgagaatttctccaccagcttctggattcgcatcccgaaatacttcaacagcattagcctgaacaacgagtatactatcatcaactgtatggagaacaacagcggttggaaggtgtctctgaactatggtgagatcatttggaccttgcaggacacccaagagatcaagcagcgcgtcgtgttcaagtactctcaaatgatcaacatttccgattacattaatcgttggatcttcgtgaccattacgaataaccgtctgaataacagcaagatttacatcaatggtcgcttgatcgatcagaaaccgattagcaacctgggtaatatccacgcaagcaacaacattatgttcaaattggacggttgccgcgatacccatcgttatatctggatcaagtatttcaacctgtttgataaagaactgaatgagaaggagatcaaagatttgtatgacaaccaatctaacagcggcattttgaaggacttctggggcgattatctgcaatacgataagccgtactatatgctgaacctggttgatccgaacaaatatgtggatgtcaataatgtgggtattcgtggttacatgtatttgaagggtccgcgtggcagcgttatgacgaccaacatttacctgaactctagcctgtaccgtggtacgaaattcatcattaagaaatatgccagcggcaacaaagataacattgtgcgtaataacgatcgtgtctacatcaacgtggtcgtgaagaataaagagtaccgtctggcgaccaacgcttcgcaggcgggtgttgagaaaattctgagcgcgttggagatccctgatgtcggtaatctgagccaagtcgtggttatgaagagcaagaacgaccagggtatcactaacaagtgcaagatgaacctgcaagacaacaatggtaacgacatcggctttattggttacaaacagttcaacaatattgctaaactggtagcgagcaattggtacaatcgtcagattgagcgcagcagccgtacttttggctgtagctgggagtttatcccggtcgatgatggttggggcgaacgtccgctgcaccatcaccatcaccatcaccatcaccattaa

SEQ ID NO: 48 - protein, 435 aa, Artificial Sequence
  Polypeptide Sequence of rHC/A Variant Y1117V F1252Y H1253K L1278F (His-tagged)
MIINTSILNLRYESNHLIDLSRYASKINIGSKVNFDPIDKNQIQLFNLESSKIEVILKNAIVYNSMYENFSTSFWIRIPKYFNSISLNNEYTIINCMENNSGWKVSLNYGEIIWTLQDTQEIKQRVVFKYSQMINISDYINRWIFVTITNNRLNNSKIYINGRLIDQKPISNLGNIHASNNIMFKLDGCRDTHRYIWIKYFNLFDKELNEKEIKDLYDNQSNSGILKDFWGDYLQYDKPYYMLNLVDPNKYVDVNNVGIRGYMYLKGPRGSVMTTNIYLNSSLYRGTKFIIKKYASGNKDNIVRNNDRVYINVVVKNKEYRLATNASQAGVEKILSALEIPDVGNLSQVVVMKSKNDQGITNKCKMNLQDNNGNDIGFIGYKQFNNIAKLVASNWYNRQIERSSRTFGCSWEFIPVDDGWGERPLHHHHHHHHHH

SEQ ID NO: 49 - DNA, 1293 bp, Artificial Sequence
  Nucleotide Sequence of rHC/A Variant Y1117V F1252Y H1253K L1278H (His-tagged)
atgatcatcaatactagcattctgaacctgcgttacgagagcaatcatctgattgatctgagccgttatgcaagcaagatcaacatcggtagcaaggtcaattttgacccgatcgataagaaccagatccagctgtttaatctggaatcgagcaaaattgaggttatcctgaaaaacgccattgtctacaactccatgtacgagaatttctccaccagcttctggattcgcatcccgaaatacttcaacagcattagcctgaacaacgagtatactatcatcaactgtatggagaacaacagcggttggaaggtgtctctgaactatggtgagatcatttggaccttgcaggacacccaagagatcaagcagcgcgtcgtgttcaagtactctcaaatgatcaacatttccgattacattaatcgttggatcttcgtgaccattacgaataaccgtctgaataacagcaagatttacatcaatggtcgcttgatcgatcagaaaccgattagcaacctgggtaatatccacgcaagcaacaacattatgttcaaattggacggttgccgcgatacccatcgttatatctggatcaagtatttcaacctgtttgataaagaactgaatgagaaggagatcaaagatttgtatgacaaccaatctaacagcggcattttgaaggacttctggggcgattatctgcaatacgataagccgtactatatgctgaacctggttgatccgaacaaatatgtggatgtcaataatgtgggtattcgtggttacatgtatttgaagggtccgcgtggcagcgttatgacgaccaacatttacctgaactctagcctgtaccgtggtacgaaattcatcattaagaaatatgccagcggcaacaaagataacattgtgcgtaataacgatcgtgtctacatcaacgtggtcgtgaagaataaagagtaccgtctggcgaccaacgcttcgcaggcgggtgttgagaaaattctgagcgcgttggagatccctgatgtcggtaatctgagccaagtcgtggttatgaagagcaagaacgaccagggtatcactaacaagtgcaagatgaacctgcaagacaacaatggtaacgacatcggctttattggttacaaacagttcaacaatattgctaaactggtagcgagcaattggtacaatcgtcagattgagcgcagcagccgtactcatggctgtagctgggagtttatcccggtcgatgatggttggggcgaacgtccgctgcaccatcaccatcaccat

SEQ ID NO: 50 - protein, 431 aa, Artificial Sequence
  Polypeptide Sequence of rHC/A Variant Y1117V F1252Y H1253K L1278H (His-tagged)
MIINTSILNLRYESNHLIDLSRYASKINIGSKVNFDPIDKNQIQLFNLESSKIEVILKNAIVYNSMYENFSTSFWIRIPKYFNSISLNNEYTIINCMENNSGWKVSLNYGEIIWTLQDTQEIKQRVVFKYSQMINISDYINRWIFVTITNNRLNNSKIYINGRLIDQKPISNLGNIHASNNIMFKLDGCRDTHRYIWIKYFNLFDKELNEKEIKDLYDNQSNSGILKDFWGDYLQYDKPYYMLNLVDPNKYVDVNNVGIRGYMYLKGPRGSVMTTNIYLNSSLYRGTKFIIKKYASGNKDNIVRNNDRVYINVVVKNKEYRLATNASQAGVEKILSALEIPDVGNLSQVVVMKSKNDQGITNKCKMNLQDNNGNDIGFIGYKQFNNIAKLVASNWYNRQIERSSRTHGCSWEFIPVDDGWGERPLHHHHHH

SEQ ID NO: 51 - protein, 1296 aa, Clostridium botulinum [sequence omitted]

SEQ ID NO: 52 - protein, 1291 aa, Clostridium botulinum
MPVTINNFNYNDPIDNNNIIMMEPPFARGTGRYYKAFKITDRIWIIPERYTFGYKPEDFNKSSGIFNRDVCEYYDPDYLNTNDKKNIFLQTMIKLFNRIKSKPLGEKLLEMIINGIPYLGDRRVPLEEFNTNIASVTVNKLISNPGEVERKKGIFANLIIFGPGPVLNENETIDIGIQNHFASREGFGGIMQMKFCPEYVSVFNNVQENKGASIFNRRGYFSDPALILMHELIHVLHGLYGIKVDDLPIVPNEKKFFMQSTDAIQAEELYTFGGQDPSIITPSTDKSIYDKVLQNFRGIVDRLNKVLVCISDPNININIYKNKFKDKYKFVEDSEGKYSIDVESFDKLYKSLMFGFTETNIAENYKIKTRASYFSDSLPPVKIKNLLDNEIYTIEEGFNISDKDMEKEYRGQNKAINKQAYEEISKEHLAVYKIQMCKSVKAPGICIDVDNEDLFFIADKNSFSDDLSKNERIEYNTQSNYIENDFPINELILDTDLISKIELPSENTESLTDFNVDVPVYEKQPAIKKIFTDENTIFQYLYSQTFPLDIRDISLTSSFDDALLFSNKVYSFFSMDYIKTANKVVEAGLFAGWVKQIVNDFVIEANKSNTMDKIADISLIVPYIGLALNVGNETAKGNFENAFEIAGASILLEFIPELLIPVVGAFLLESYIDNKNKIIKTIDNALTKRNEKWSDMYGLIVAQWLSTVNTQFYTIKEGMYKALNYQAQALEEIIKYRYNIYSEKEKSNINIDFNDINSKLNEGINQAIDNINNFINGCSVSYLMKKMIPLAVEKLLDFDNTLKKNLLNYIDENKLYLIGSAEYEKSKVNKYLKTIMPFDLSIYTNDTILIEMFNKYNSEILNNIILNLRYKDNNLIDLSGYGAKVEVYDGVELNDKNQFKLTSSANSKIRVTQNQNIIFNSVFLDFSVSFWIRIPKYKNDGIQNYIHNEYTIINCMKNNSGWKISIRGNRIIWTLIDINGKTKSVFFEYNIREDISEYINRWFFVTITNNLNNAKIYINGKLESNTDIKDIREVIANGEIIFKLDGDIDRTQFIWMKYFSIFNTELSQSNIEERYKIQSYSEYLKDFWGNPLMYNKEYYMFNAGNKNSYIKLKKDSPVGEILTRSKYNQNSKYINYRDLYIGEKFIIRRKSNSQSINDDIVRKEDYIYLDFFNLNQEWRVYTYKYFKKEEEKLFLAPISDSDEFYNTIQIKEYDEQPTYSCQLLFKKDEESTDEIGLIGIHRFYESGIVFEEYKDYFCISKWYLKEVKRKPYNLKLGCNWQFIPKDEGWTE

SEQ ID NO: 53 - protein, 1291 aa, Clostridium botulinum
MPITINNFNYSDPVDNKNILYLDTHLNTLANEPEKAFRITGNIWVIPDRFSRNSNPNLNKPPRVTSPKSGYYDPNYLSTDSDKDPFLKEIIKLFKRINSREIGEELIYRLSTDIPFPGNNNTPINTFDFDVDFNSVDVKTRQGNNWVKTGSINPSVIITGPRENIIDPETSTFKLTNNTFAAQEGFGALSIISISPRFMLTYSNATNDVGEGRFSKSEFCMDPILILMHELNHAMHNLYGIAIPNDQTISSVTSNIFYSQYNVKLEYAEIYAFGGPTIDLIPKSARKYFEEKALDYYRSIAKRLNSITTANPSSFNKYIGEYKQKLIRKYRFVVESSGEVTVNRNKFVELYNELTQIFTEFNYAKIYNVQNRKIYLSNVYTPVTANILDDNVYDIQNGFNIPKSNLNVLFMGQNLSRNPALRKVNPENMLYLFTKFCHKAIDGRSLYNKTLDCRELLVKNTDLPFIGDISDVKTDIFLRKDINEETEVIYYPDNVSVDQVILSKNTSEHGQLDLLYPSIDSESEILPGENQVFYDNRTQNVDYLNSYYYLESQKLSDNVEDFTFTRSIEEALDNSAKVYTYFPTLANKVNAGVQGGLFLMWANDVVEDFTTNILRKDTLDKISDVSAIIPYIGPALNISNSVRRGNFTEAFAVTGVTILLEAFPEFTIPALGAFVIYSKVQERNEIIKTIDNCLEQRIKRWKDSYEWMMGTWLSRIITQFNNISYQMYDSLNYQAGAIKAKIDLEYKKYSGSDKENIKSQVENLKNSLDVKISEAMNNINKFIRECSVTYLFKNMLPKVIDELNEFDRNTKAKLINLIDSHNIILVGEVDKLKAKVNNSFQNTIPFNIFSYTNNSLLKDIINEYFNNINDSKILSLQNRKNTLVDTSGYNAEVSEEGDVQLNPIFPFDFKLGSSGEDRGKVIVTQNENIVYNSMYESFSISFWIRINKWVSNLPGYTIIDSVKNNSGWSIGIISNFLVFTLKQNEDSEQSINFSYDISNNAPGYNKWFFVTVTNNMMGNMKIYINGKLIDTIKVKELTGINFSKTITFEINKIPDTGLITSDSDNINMWIRDFYIFAKELDGKDINILFNSLQYTNVVKDYWGNDLRYNKEYYMVNIDYLNRYMYANSRQIVFNTRRNNNDFNEGYKIIIKRIRGNTNDTRVRGGDILYFDMTINNKAYNLFMKNETMYADNHSTEDIYAIGLREQTKDINDNIIFQIQPMNNTYYYASQIFKSNFNGENISGICSIGTYRFRLGGDWYRHNYLVPTVKQGNYASLLESTSTHWGFVPVSE

SEQ ID NO: 54 - protein, 1276 aa, Clostridium botulinum
MTWPVKDFNYSDPVNDNDILYLRIPQNKLITTPVKAFMITQNIWVIPERFSSDTNPSLSKPPRPTSKYQSYYDPSYLSTDEQKDTFLKGIIKLFKRINERDIGKKLINYLVVGSPFMGDSSTPEDTFDFTRHTTNIAVEKFENGSWKVTNIITPSVLIFGPLPNILDYTASLTLQGQQSNPSFEGFGTLSILKVAPEFLLTFSDVTSNQSSAVLGKSIFCMDPVIALMHELTHSLHQLYGINIPSDKRIRPQVSEGFFSQDGPNVQFEELYTFGGLDVEIIPQIERSQLREKALGHYKDIAKRLNNINKTIPSSWISNIDKYKKIFSEKYNFDKDNTGNFVVNIDKFNSLYSDLTNVMSEVVYSSQYNVKNRTHYFSRHYLPVFANILDDNIYTIRDGFNLTNKGFNIENSGQNIERNPALQKLSSESVVDLFTKVCLRLTKNSRDDSTCIKVKNNRLPYVADKDSISQEIFENKIITDETNVQNYSDKFSLDESILDGQVPINPEIVDPLLPNVNMEPLNLPGEEIVFYDDITKYVDYLNSYYYLESQKLSNNVENITLTTSVEEALGYSNKIYTFLPSLAEKVNKGVQAGLFLNWANEVVEDFTTNIMKKDTLDKISDVSVIIPYIGPALNIGNSALRGNFNQAFATAGVAFLLEGFPEFTIPALGVFTFYSSIQEREKIIKTIENCLEQRVKRWKDSYQWMVSNWLSRITTQFNHINYQMYDSLSYQADAIKAKIDLEYKKYSGSDKENIKSQVENLKNSLDVKISEAMNNINKFIRECSVTYLFKNMLPKVIDELNKFDLRTKTELINLIDSHNIILVGEVDRLKAKVNESFENTMPFNIFSYTNNSLLKDIINEYFNSINDSKILSLQNKKNALVDTSGYNAEVRVGDNVQLNTIYTNDFKLSSSGDKIIVNLNNNILYSAIYENSSVSFWIKISKDLTNSHNEYTIINSIEQNSGWKLCIRNGNIEWILQDVNRKYKSLIFDYSESLSHTGYTNKWFFVTITNNIMGYMKLYINGELKQSQKIEDLDEVKLDKTIVFGIDENIDENQMLWIRDFNIFSKELSNEDINIVYEGQILRNVIKDYWGNPLKFDTEYYIINDNYIDRYIAPESNVLVLVQYPDRSKLYTGNPITIKSVSDKNPYSRILNGDNIILHMLYNSRKYMIIRDTDTIYATQGGECSQNCVYALKLQSNLGNYGIGIFSIKNIVSKNKYCSQIFSSFRENTMLLADIYKPWRFSFKNAYTPVAVTNYETKLLSTSSFWKFISRDPGWVE

SEQ ID NO: 55 - protein, 1251 aa, Clostridium botulinum
MPKINSFNYNDPVNDRTILYIKPGGCQEFYKSFNIMKNIWIIPERNVIGTTPQDFHPPTSLKNGDSSYYDPNYLQSDEEKDRFLKIVTKIFNRINNNLSGGILLEELSKANPYLGNDNTPDNQFHIGDASAVEIKFSNGSQDILLPNVIIMGAEPDLFETNSSNISLRNNYMPSNHRFGSIAIVTFSPEYSFRFNDNCMNEFIQDPALTLMHELIHSLHGLYGAKGITTKYTITQKQNPLITNIRGTNIEEFLTFGGTDLNIITSAQSNDIYTNLLADYKKIASKLSKVQVSNPLLNPYKDVFEAKYGLDKDASGIYSVNINKFNDIFKKLYSFTEFDLRTKFQVKCRQTYIGQYKYFKLSNLLNDSIYNISEGYNINNLKVNFRGQNANLNPRIITPITGRGLVKKIIRFCKNIVSVKGIRKSICIEINNGELFFVASENSYNDDNINTPKEIDDTVTSNNNYENDLDQVILNFNSESAPGLSDEKLNLTIQNDAYIPKYDSNGTSDIEQHDVNELNVFFYLDAQKVPEGENNVNLTSSIDTALLEQPKIYTFFSSEFINNVNKPVQAALFVSWIQQVLVDFTTEANQKSTVDKIADISIVVPYIGLALNIGNEAQKGNFKDALELLGAGILLEFEPELLIPTILVFTIKSFLGSSDNKNKVIKAINNALKERDEKWKEVYSFIVSNWMTKINTQFNKRKEQMYQALQNQVNAIKTIIESKYNSYTLEEKNELTNKYDIKQIENELNQKVSIAMNNIDRFLTESSISYLMKIINEVKINKLREYDENVKTYLLNYIIQHGSILGESQQELNSMVTDTLNNSIPFKLSSYTDDKILISYFNKFFKRIKSSSVLNMRYKNDKYVDTSGYDSNININGDVYKYPTNKNQFGIYNDKLSEVNISQNDYIIYDNKYKNFSISFWVRIPNYDNKIVNVNNEYTIINCMRDNNSGWKVSLNHNEIIWTFEDNRGINQKLAFNYGNANGISDYINKWIFVTITNDRLGDSKLYINGNLIDQKSILNLGNIHVSDNILFKIVNCSYTRYIGIRYFNIFDKELDETEIQTLYSNEPNTNILKDFWGNYLLYDKEYYLLNVLKPNNFIDRRKDSTLSINNIRSTILLANRLYSGIKVKIQRVNNSSTNDNLVRKNDQVYINFVASKTHLFPLYADTATTNKEKTIKISSSGNRFNQVVVMNSVGNCTMNFKNNNGNNIGLLGFKADTVVASTWYYTHMRDHTNSNGCFWNFISEEHGWQEK

SEQ ID NO: 56 - protein, 1278 aa, Clostridium botulinum
MPVVINSFNYNDPVNDDTILYMQIPYEEKSKKYYKAFEIMRNVWIIPERNTIGTDPSDFDPPASLENGSSAYYDPNYLTTDAEKDRYLKTTIKLFKRINSNPAGEVLLQEISYAKPYLGNEHTPINEFHPVTRTTSVNIKSSTNVKSSIILNLLVLGAGPDIFENSSYPVRKLMDSGGVYDPSNDGFGSINIVTFSPEYEYTFNDISGGYNSSTESFIADPAISLAHELIHALHGLYGARGVTYKETIKVKQAPLMIAEKPIRLEEFLTFGGQDLNIITSAMKEKIYNNLLANYEKIATRLSRVNSAPPEYDINEYKDYFQWKYGLDKNADGSYTVNENKFNEIYKKLYSFTEIDLANKFKVKCRNTYFIKYGFLKVPNLLDDDIYTVSEGFNIGNLAVNNRGQNIKLNPKIIDSIPDKGLVEKIVKFCKSVIPRKGTKAPPRLCIRVNNRELFFVASESSYNENDINTPKEIDDTTNLNNNYRNNLDEVILDYNSETIPQISNQTLNTLVQDDSYVPRYDSNGTSEIEEHNVVDLNVFFYLHAQKVPEGETNISLTSSIDTALSEESQVYTFFSSEFINTINKPVHAALFISWINQVIRDFTTEATQKSTFDKIADISLVVPYVGLALNIGNEVQKENFKEAFELLGAGILLEFVPELLIPTILVFTIKSFIGSSENKNKIIKAINNSLMERETKWKEIYSWIVSNWLTRINTQFNKRKEQMYQALQNQVDAIKTVIEYKYNNYTSDERNRLESEYNINNIREELNKKVSLAMENIERFITESSIFYLMKLINEAKVSKLREYDEGVKEYLLDYISEHRSILGNSVQELNDLVTSTLNNSIPFELSSYTNDKILILYFNKLYKKIKDNSILDMRYENNKFIDISGYGSNISINGDVYIYSTNRNQFGIYSSKPSEVNIAQNNDIIYNGRYQNFSISFWVRIPKYFNKVNLNNEYTIIDCIRNNNSGWKISLNYNKIIWTLQDTAGNNQKLVFNYTQMISISDYINKWIFVTITNNRLGNSRIYINGNLIDEKSISNLGDIHVSDNILFKIVGCNDTRYVGIRYFKVFDTELGKTEIETLYSDEPDPSILKDFWGNYLLYNKRYYLLNLLRTDKSITQNSNFLNINQQRGVYQKPNIFSNTRLYTGVEVIIRKNGSTDISNTDNFVRKNDLAYINVVDRDVEYRLYADISIAKPEKIIKLIRTSNSNNSLGQIIVMDSIGNNCTMNFQNNNGGNIGLLGFHSNNLVASSWYYNNIRKNTSSNGCFWSFISKEHGWQEN

SEQ ID NO: 57 - protein, 1297 aa, Clostridium botulinum
  misc_feature (7)..(7): Xaa can be any naturally occurring amino acid
MPVNIKXFNYNDPINNDDIIMMEPFNDPGPGTYYKAFRIIDRIWIVPERFTYGFQPDQFNASTGVFSKDVYEYYDPTYLKTDAEKDKFLKTMIKLFNRINSKPSGQRLLDMIVDAIPYLGNASTPPDKFAANVANVSINKKIIQPGAEDQIKGLMTNLIIFGPGPVLSDNFTDSMIMNGHSPISEGFGARMMIRFCPSCLNVFNNVQENKDTSIFSRRAYFADPALTLMHELIHVLHGLYGIKISNLPITPNTKEFFMQHSDPVQAEELYTFGGHDPSVISPSTDMNIYNKALQNFQDIANRLNIVSSAQGSGIDISLYKQIYKNKYDFVEDPNGKYSVDKDKFDKLYKALMFGFTETNLAGEYGIKTRYSYFSEYLPPIKTEKLLDNTIYTQNEGFNIASKNLKTEFNGQNKAVNKEAYEEISLEHLVIYRIAMCKPVMYKNTGKSEQCIIVNNEDLFFIANKDSFSKDLAKAETIAYNTQNNTIENNFSIDQLILDNDLSSGIDLPNENTEPFTNFDDIDIPVYIKQSALKKIFVDGDSLFEYLHAQTFPSNIENLQLTNSLNDALRNNNKVYTFFSTNLVEKANTVVGASLFVNWVKGVIDDFTSESTQKSTIDKVSDVSIIIPYIGPALNVGNETAKENFKNAFEIGGAAILMEFIPELIVPIVGFFTLESYVGNKGHIIMTISNALKKRDQKWTDMYGLIVSQWLSTVNTQFYTIKERMYNALNNQSQAIEKIIEDQYNRYSEEDKMNINIDFNDIDFKLNQSINLAINNIDDFINQCSISYLMNRMIPLAVKKLKDFDDNLKRDLLEYIDTNELYLLDEVNILKSKVNRHLKDSIPFDLSLYTKDTILIQVFNNYISNISSNAILSLSYRGGRLIDSSGYGATMNVGSDVIFNDIGNGQFKLNNSENSNITAHQSKFVVYDSMFDNFSINFWVRTPKYNNNDIQTYLQNEYTIISCIKNDSGWKVSIKGNRIIWTLIDVNAKSKSIFFEYSIKDNISDYINKWFSITITNDRLGNANIYINGSLKKSEKILNLDRINSSNDIDFKLINCTDTTKFVWIKDFNIFGRELNATEVSSLYWIQSSTNTLKDFWGNPLRYDTQYYLFNQGMQNIYIKYFSKASMGETAPRTNFNNAAINYQNLYLGLRFIIKKASNSRNINNDNIVREGDYIYLNIDNISDESYRVYVLVNSKEIQTQLFLAPINDDPTFYDVLQIKKYYEKTTYNCQILCEKDTKTFGLFGIGKFVKDYGYVWDTYDNYFCISQWYLRRISENINKLRLGCNWQFIPVDEGWTE

SEQ ID NO: 58 - protein, 1315 aa, Clostridium tetani
MPITINNFRYSDPVNNDTIIMMEPPYCKGLDIYYKAFKITDRIWIVPERYEFGTKPEDFNPPSSLIEGASEYYDPNYLRTDSDKDRFLQTMVKLFNRIKNNVAGEALLDKIINAIPYLGNSYSLLDKFDTNSNSVSFNLLEQDPSGATTKSAMLTNLIIFGPGPVLNKNEVRGIVLRVDNKNYFPCRDGFGSIMQMAFCPEYVPTFDNVIENITSLTIGKSKYFQDPALLLMHELIHVLHGLYGMQVSSHEIIPSKQEIYMQHTYPISAEELFTFGGQDANLISIDIKNDLYEKTLNDYKAIANKLSQVTSCNDPNIDIDSYKQIYQQKYQFDKDSNGQYIVNEDKFQILYNSIMYGFTEIELGKKFNIKTRLSYFSMNHDPVKIPNLLDDTIYNDTEGFNIESKDLKSEYKGQNMRVNTNAFRNVDGSGLVSKLIGLCKKIIPPTNIRENLYNRTASLTDLGGELCIKIKNEDLTFIAEKNSFSEEPFQDEIVSYNTKNKPLNFNYSLDKIIVDYNLQSKITLPNDRTTPVTKGIPYAPEYKSNAASTIEIHNIDDNTIYQYLYAQKSPTTLQRITMTNSVDDALINSTKIYSYFPSVISKVNQGAQGILFLQWVRDIIDDFTNESSQKTTIDKISDVSTIVPYIGPALNIVKQGYEGNFIGALETTGVVLLLEYIPEITLPVIAALSIAESSTQKEKIIKTIDNFLEKRYEKWIEVYKLVKAKWLGTVNTQFQKRSYQMYRSLEYQVDAIKKIIDYEYKIYSGPDKEQIADEINNLKNKLEEKANKAMININIFMRESSRSFLVNQMINEAKKQLLEFDTQSKNILMQYIKANSKFIGITELKKLESKINKVFSTPIPFSYSKNLDCWVDNEEDIDVILKKSTILNLDINNDIISDISGFNSSVITYPDAQLVPGINGKAIHLVNNESSEVIVHKAMDIEYNDMFNNFTVSFWLRVPKVSASHLEQYGTNEYSIISSMKKHSLSIGSGWSVSLKGNNLIWTLKDSAGEVRQITFRDLPDKFNAYLANKWVFITITNDRLSSANLYINGVLMGSAEITGLGAIREDNNITLKLDRCNNNNQYVSIDKFRIFCKALNPKEIEKLYTSYLSITFLRDFWGNPLRYDTEYYLIPVASSSKDVQLKNITDYMYLTNAPSYTNGKLNIYYRRLYNGLKFIIKRYTPNNEIDSFVKSGDFIKLYVSYNNNEHIVGYPKDGNAFNNLDRILRVGYNAPGIPLYKKMEAVKLRDLKTYSVQLKLYDDKNASLGLVGTHNGQIGNDPNRDILIASNWYFNHLKDKILGCDWYFVPTDEGWTND

SEQ ID NO: 59 - protein, 1306 aa, Clostridium botulinum
MKLEINKFNYNDPIDGINVITMRPPRHSDKINKGKGPFKAFQVIKNIWIVPERYNFTNNTNDLNIPSEPIMEADAIYNPNYLNTPSEKDEFLQGVIKVLERIKSKPEGEKLLELISSSIPLPLVSNGALTLSDNETIAYQENNNIVSNLQANLVIYGPGPDIANNATYGLYSTPISNGEGTLSEVSFSPFYLKPFDESYGNYRSLVNIVNKFVKREFAPDPASTLMHELVHVTHNLYGISNRNFYYNFDTGKIETSRQQNSLIFEELLTFGGIDSKAISSLIIKKIIETAKNNYTTLISERLNTVTVENDLLKYIKNKIPVQGRLGNFKLDTAEFEKKLNTILFVLNESNLAQRFSILVRKHYLKERPIDPIYVNILDDNSYSTLEGFNISSQGSNDFQGQLLESSYFEKIESNALRAFIKICPRNGLLYNAIYRNSKNYLNNIDLEDKKTTSKTNVSYPCSLLNGCIEVENKDLFLISNKDSLNDINLSEEKIKPETTVFFKDKLPPQDITLSNYDFTEANSIPSISQQNILERNEELYEPIRNSLFEIKTIYVDKLTTFHFLEAQNIDESIDSSKIRVELTDSVDEALSNPNKVYSPFKNMSNTINSIETGITSTYIFYQWLRSIVKDFSDETGKIDVIDKSSDTLAIVPYIGPLLNIGNDIRHGDFVGAIELAGITALLEYVPEFTIPILVGLEVIGGELAREQVEAIVNNALDKRDQKWAEVYNITKAQWWGTIHLQINTRLAHTYKALSRQANAIKMNMEFQLANYKGNIDDKAKIKNAISETEILLNKSVEQAMKNTEKFMIKLSNSYLTKEMIPKVQDNLKNFDLETKKTLDKFIKEKEDILGTNLSSSLRRKVSIRLNKNIAFDINDIPFSEFDDLINQYKNEIEDYEVLNLGAEDGKIKDLSGTTSDINIGSDIELADGRENKAIKIKGSENSTIKIAMNKYLRFSATDNFSISFWIKHPKPTNLLNNGIEYTLVENFNQRGWKISIQDSKLIWYLRDHNNSIKIVTPDYIAFNGWNLITITNNRSKGSIVYVNGSKIEEKDISSIWNTEVDDPIIFRLKNNRDTQAFTLLDQFSIYRKELNQNEVVKLYNYYFNSNYIRDIWGNPLQYNKKYYLQTQDKPGKGLIREYWSSFGYDYVILSDSKTITFPNNIRYGALYNGSKVLIKNSKKLDGLVRNKDFIQLEIDGYNMGISADRFNEDTNYIGTTYGTTHDLTTDFEIIQRQEKYRNYCQLKTPYNIFHKSGLMSTETSKPTFHDYRDWVYSSAWYFQNYENLNLRKHTKTNWYFIPKDEGWDED

SEQ ID NO: 60 - DNA, 3888 bp, Artificial Sequence
  Nucleotide Sequence of mrBoNT/A
atgccattcgtcaacaagcaattcaactacaaagacccagtcaacggcgtcgacatcgcatacatcaagattccgaacgccggtcaaatgcagccggttaaggcttttaagatccacaacaagatttgggttatcccggagcgtgacaccttcacgaacccggaagaaggcgatctgaacccgccaccggaagcgaagcaagtccctgtcagctactacgattcgacgtacctgagcacggataacgaaaaagataactacctgaaaggtgtgaccaagctgttcgaacgtatctacagcacggatctgggtcgcatgctgctgactagcattgttcgcggtatcccgttctggggtggtagcacgattgacaccgaactgaaggttatcgacactaactgcattaacgttattcaaccggatggtagctatcgtagcgaagagctgaatctggtcatcattggcccgagcgcagacattatccaattcgagtgcaagagctttggtcacgaggttctgaatctgacccgcaatggctatggtagcacccagtacattcgtttttcgccggattttaccttcggctttgaagagagcctggaggttgataccaatccgttgctgggtgcgggcaaattcgctaccgatccggctgtcacgctggcccatgaactgatccacgcaggccaccgcctgtacggcattgccatcaacccaaaccgtgtgttcaaggttaatacgaatgcatactacgagatgagcggcctggaagtcagcttcgaagaactgcgcaccttcggtggccatgacgctaaattcattgacagcttgcaagagaatgagttccgtctgtactactataacaaattcaaagacattgcaagcacgttgaacaaggccaaaagcatcgttggtactaccgcgtcgttgcagtatatgaagaatgtgtttaaagagaagtacctgctgtccgaggatacctccggcaagtttagcgttgataagctgaagtttgacaaactgtacaagatgctgaccgagatttacaccgaggacaactttgtgaaattcttcaaagtgttgaatcgtaaaacctatctgaattttgacaaagcggttttcaagattaacatcgtgccgaaggtgaactacaccatctatgacggttttaacctgcgtaacaccaacctggcggcgaactttaacggtcagaatacggaaatcaacaacatgaatttcacgaagttgaagaacttcacgggtctgttcgagttctataagctgctgtgcgtgcgcggtatcatcaccagcaaaaccaaaagcctggacaaaggctacaacaaggcgctgaatgacctgtgcattaaggtaaacaattgggatctgttcttttcgccatccgaagataattttaccaacgacctgaacaagggtgaagaaatcaccagcgatacgaatattgaagcagcggaagagaatatcagcctggatctgatccagcagtactatctgacctttaacttcgacaatgaaccggagaacattagcattgagaatctgagcagcgacattatcggtcagctggaactgatgccgaatatcgaacgtttcccgaacggcaaaaagtacgagctggacaagtacactatgttccattacctgcgtgcacaggagtttgaacacggtaaaagccgtatcgcgctgaccaacagcgttaacgaggccctgctgaacccgagccgtgtctataccttcttcagcagcgactatgttaagaaagtgaacaaagccactgaggccgcgatgttcctgggctgggtggaacagctggtatatgacttcacggacgagacgagcgaagtgagcactaccgacaaaattgctgatattaccatcattatcccgtatattggtccggcactgaacattggcaacatgctgtacaaagacgattttgtgggtgccctgatcttctccggtgccgtgattctgctggagttcattccggagattgcgatcccggtgttgggtaccttcgcgctggtgtcctacatcgcgaataaggttctgacggttcagaccatcgataacgcgctgtcgaaacgtaatgaaaaatgggacgaggtttacaaatacattgttacgaattggctggcgaaagtcaatacccagatcgacctgatccgtaagaaaatgaaagaggcgctggagaatcaggcggaggccaccaaagcaattatcaactaccaatacaaccagtacacggaagaagagaagaataacattaacttcaatatcgatgatttgagcagcaagctgaatgaatctatcaacaaagcgatgatcaatatcaacaagtttttgaatcagtgtagcgtttcgtacctgatgaatagcatgattccgtatggcgtcaaacgtctggaggacttcgacgccagcctgaaagatgcgttgctgaaatacatttacgacaatcgtggtacgctgattggccaagttgaccgcttgaaagacaaagttaacaataccctgagcaccgacatcccatttcaactgagcaagtatgttgataatcaacgtctgttgagcactttcaccgagtatatcaaaaacatcatcaatactagcattctgaacctgcgttacgagagcaagcatctgattgatctgagccgttatgctagcaagatcaacatcggtagcaaggtcaattttgacccgatcgataagaaccagatccagctgtttaatctggaatcgagcaaaattgaggttatcctgaaaaaggccattgtctacaactccatgtacgagaatttctccaccagcttctggattcgcatcccgaaatacttcaacaagattagcctgaacaacgagtatactatcatcaactgtatggagaacaacagcggttggaaggtgtctctgaactatggtgagatcatttggaccttgcaggacaccaaagagatcaagcagcgcgtcgtgttcaagtactctcaaatgatcaacatttccgattacattaatcgttggatcttcgtgaccattacgaataaccgtctgaataagagcaagatttacatcaatggtcgcttgatcgatcagaaaccgattagcaacctgggtaatatccacgcaagcaacaagattatgttcaaattggacggttgccgcgatacccatcgttatatctggatcaagtatttcaacctgtttgataaagaactgaatgagaaggagatcaaagatttgtatgacaaccaatctaacagcggcattttgaaggacttctggggcgattatctgcaatacgataagccgtactatatgctgaacctgtatgatccgaacaaatatgtggatgtcaataatgtgggtattcgtggttacatgtatttgaagggtccgcgtggcagcgttatgacgaccaacatttacctgaactctagcctgtaccgtggtacgaaattcatcattaagaaatatgccagcggcaacaaagataacattgtgcgtaataacgatcgtgtctacatcaacgtggtcgtgaagaataaagagtaccgtctggcgaccaacgcttcgcaggcgggtgttgagaaaattctgagcgcgttggagatccctgatgtcggtaatctgagccaagtcgtggttatgaagagcaagaacgacaagggtatcactaacaagtgcaagatgaacctgcaagacaacaatggtaacgacatcggctttattggtttccaccagttcaacaatattgctaaactggtagcgagcaattggtacaatcgtcagattgagcgcagcagccgtactttgggctgtagctgggagtttatcccggtcgatgatggttggggcgaacgtccgctg

SEQ ID NO: 61 - protein, 1296 aa, Artificial Sequence
  Polypeptide Sequence of mrBoNT/A
MPFVNKQFNYKDPVNGVDIAYIKIPNAGQMQPVKAFKIHNKIWVIPERDTFTNPEEGDLNPPPEAKQVPVSYYDSTYLSTDNEKDNYLKGVTKLFERIYSTDLGRMLLTSIVRGIPFWGGSTIDTELKVIDTNCINVIQPDGSYRSEELNLVIIGPSADIIQFECKSFGHEVLNLTRNGYGSTQYIRFSPDFTFGFEESLEVDTNPLLGAGKFATDPAVTLAHELIHAGHRLYGIAINPNRVFKVNTNAYYEMSGLEVSFEELRTFGGHDAKFIDSLQENEFRLYYYNKFKDIASTLNKAKSIVGTTASLQYMKNVFKEKYLLSEDTSGKFSVDKLKFDKLYKMLTEIYTEDNFVKFFKVLNRKTYLNFDKAVFKINIVPKVNYTIYDGFNLRNTNLAANFNGQNTEINNMNFTKLKNFTGLFEFYKLLCVRGIITSKTKSLDKGYNKALNDLCIKVNNWDLFFSPSEDNFTNDLNKGEEITSDTNIEAAEENISLDLIQQYYLTFNFDNEPENISIENLSSDIIGQLELMPNIERFPNGKKYELDKYTMFHYLRAQEFEHGKSRIALTNSVNEALLNPSRVYTFFSSDYVKKVNKATEAAMFLGWVEQLVYDFTDETSEVSTTDKIADITIIIPYIGPALNIGNMLYKDDFVGALIFSGAVILLEFIPEIAIPVLGTFALVSYIANKVLTVQTIDNALSKRNEKWDEVYKYIVTNWLAKVNTQIDLIRKKMKEALENQAEATKAIINYQYNQYTEEEKNNINFNIDDLSSKLNESINKAMININKFLNQCSVSYLMNSMIPYGVKRLEDFDASLKDALLKYIYDNRGTLIGQVDRLKDKVNNTLSTDIPFQLSKYVDNQRLLSTFTEYIKNIINTSILNLRYESKHLIDLSRYASKINIGSKVNFDPIDKNQIQLFNLESSKIEVILKKAIVYNSMYENFSTSFWIRIPKYFNKISLNNEYTIINCMENNSGWKVSLNYGEIIWTLQDTKEIKQRVVFKYSQMINISDYINRWIFVTITNNRLNKSKIYINGRLIDQKPISNLGNIHASNKIMFKLDGCRDTHRYIWIKYFNLFDKELNEKEIKDLYDNQSNSGILKDFWGDYLQYDKPYYMLNLYDPNKYVDVNNVGIRGYMYLKGPRGSVMTTNIYLNSSLYRGTKFIIKKYASGNKDNIVRNNDRVYINVVVKNKEYRLATNASQAGVEKILSALEIPDVGNLSQVVVMKSKNDKGITNKCKMNLQDNNGNDIGFIGFHQFNNIAKLVASNWYNRQIERSSRTLGCSWEFIPVDDGWGERPL

SEQ ID NO: 62 - protein, 1296 aa, Clostridium botulinum
MPFVNKQFNYKDPVNGVDIAYIKIPNAGQMQPVKAFKIHNKIWVIPERDTFTNPEEGDLNPPPEAKQVPVSYYDSTYLSTDNEKDNYLKGVTKLFERIYSTDLGRMLLTSIVRGIPFWGGSTIDTELKVIDTNCINVIQPDGSYRSEELNLVIIGPSADIIQFECKSFGHEVLNLTRNGYGSTQYIRFSPDFTFGFEESLEVDTNPLLGAGKFATDPAVTLAHELIHAGHRLYGIAINPNRVFKVNTNAYYEMSGLEVSFEELRTFGGHDAKFIDSLQENEFRLYYYNKFKDIASTLNKAKSIVGTTASLQYMKNVFKEKYLLSEDTSGKFSVDKLKFDKLYKMLTEIYTEDNFVKFFKVLNRKTYLNFDKAVFKINIVPKVNYTIYDGFNLRNTNLAANFNGQNTEINNMNFTKLKNFTGLFEFYKLLCVRGIITSKTKSLDKGYNKALNDLCIKVNNWDLFFSPSEDNFTNDLNKGEEITSDTNIEAAEENISLDLIQQYYLTFNFDNEPENISIENLSSDIIGQLELMPNIERFPNGKKYELDKYTMFHYLRAQEFEHGKSRIALTNSVNEALLNPSRVYTFFSSDYVKKVNKATEAAMFLGWVEQLVYDFTDETSEVSTTDKIADITIIIPYIGPALNIGNMLYKDDFVGALIFSGAVILLEFIPEIAIPVLGTFALVSYIANKVLTVQTIDNALSKRNEKWDEVYKYIVTNWLAKVNTQIDLIRKKMKEALENQAEATKAIINYQYNQYTEEEKNNINFNIDDLSSKLNESINKAMININKFLNQCSVSYLMNSMIPYGVKRLEDFDASLKDALLKYIYDNRGTLIGQVDRLKDKVNNTLSTDIPFQLSKYVDNQRLLSTFTEYIKNIINTSILNLRYESNHLIDLSRYASKINIGSKVNFDPIDKNQIQLFNLESSKIEVILKNAIVYNSMYENFSTSFWIRIPKYFNSISLNNEYTIINCMENNSGWKVSLNYGEIIWTLQDTQEIKQRVVFKYSQMINISDYINRWIFVTITNNRLNNSKIYINGRLIDQKPISNLGNIHASNNIMFKLDGCRDTHRYIWIKYFNLFDKELNEKEIKDLYDNQSNSGILKDFWGDYLQYDKPYYMLNLYDPNKYVDVNNVGIRGYMYLKGPRGSVMTTNIYLNSSLYRGTKFIIKKYASGNKDNIVRNNDRVYINVVVKNKEYRLATNASQAGVEKILSALEIPDVGNLSQVVVMKSKNDQGITNKCKMNLQDNNGNDIGFIGFHQFNNIAKLVASNWYNRQIERSSRTLGCSWEFIPVDDGWGERPL

SEQ ID NO: 63 - protein, 1304 aa, Artificial Sequence
  Polypeptide Sequence of mrBoNT/AB
MPFVNKQFNYKDPVNGVDIAYIKIPNAGQMQPVKAFKIHNKIWVIPERDTFTNPEEGDLNPPPEAKQVPVSYYDSTYLSTDNEKDNYLKGVTKLFERIYSTDLGRMLLTSIVRGIPFWGGSTIDTELKVIDTNCINVIQPDGSYRSEELNLVIIGPSADIIQFECKSFGHEVLNLTRNGYGSTQYIRFSPDFTFGFEESLEVDTNPLLGAGKFATDPAVTLAHELIHAGHRLYGIAINPNRVFKVNTNAYYEMSGLEVSFEELRTFGGHDAKFIDSLQENEFRLYYYNKFKDIASTLNKAKSIVGTTASLQYMKNVFKEKYLLSEDTSGKFSVDKLKFDKLYKMLTEIYTEDNFVKFFKVLNRKTYLNFDKAVFKINIVPKVNYTIYDGFNLRNTNLAANFNGQNTEINNMNFTKLKNFTGLFEFYKLLCVRGIITSKTKSLDKGYNKALNDLCIKVNNWDLFFSPSEDNFTNDLNKGEEITSDTNIEAAEENISLDLIQQYYLTFNFDNEPENISIENLSSDIIGQLELMPNIERFPNGKKYELDKYTMFHYLRAQEFEHGKSRIALTNSVNEALLNPSRVYTFFSSDYVKKVNKATEAAMFLGWVEQLVYDFTDETSEVSTTDKIADITIIIPYIGPALNIGNMLYKDDFVGALIFSGAVILLEFIPEIAIPVLGTFALVSYIANKVLTVQTIDNALSKRNEKWDEVYKYIVTNWLAKVNTQIDLIRKKMKEALENQAEATKAIINYQYNQYTEEEKNNINFNIDDLSSKLNESINKAMININKFLNQCSVSYLMNSMIPYGVKRLEDFDASLKDALLKYIYDNRGTLIGQVDRLKDKVNNTLSTDIPFQLSKYVDNQRLLSTFTEYIKNILNNIILNLRYKDNNLIDLSGYGAKVEVYDGVELNDKNQFKLTSSANSKIRVTQNQNIIFNSVFLDFSVSFWIRIPKYKNDGIQNYIHNEYTIINCMKNNSGWKISIRGNRIIWTLIDINGKTKSVFFEYNIREDISEYINRWFFVTITNNLNNAKIYINGKLESNTDIKDIREVIANGEIIFKLDGDIDRTQFIWMKYFSIFNTELSQSNIEERYKIQSYSEYLKDFWGNPLMYNKEYYMFNAGNKNSYIKLKKDSPVGEILTRSKYNQNSKYINYRDLYIGEKFIIRRKSNSQSINDDIVRKEDYIYLDFFNLNQEWRVYTYKYFKKEEMKLFLAPIYDSDEFYNTIQIKEYDEQPTYSCQLLFKKDEESTDEIGLIGIHRFYESGIVFEEYKDYFCISKWYLKEVKRKPYNLKLGCNWQFIPKDEGWTE

SEQ ID NO: 64 - protein, 1304 aa, Artificial Sequence
  Polypeptide Sequence of mrBoNT/AB(0)
MPFVNKQFNYKDPVNGVDIAYIKIPNAGQMQPVKAFKIHNKIWVIPERDTFTNPEEGDLNPPPEAKQVPVSYYDSTYLSTDNEKDNYLKGVTKLFERIYSTDLGRMLLTSIVRGIPFWGGSTIDTELKVIDTNCINVIQPDGSYRSEELNLVIIGPSADIIQFECKSFGHEVLNLTRNGYGSTQYIRFSPDFTFGFEESLEVDTNPLLGAGKFATDPAVTLAHQLIYAGHRLYGIAINPNRVFKVNTNAYYEMSGLEVSFEELRTFGGHDAKFIDSLQENEFRLYYYNKFKDIASTLNKAKSIVGTTASLQYMKNVFKEKYLLSEDTSGKFSVDKLKFDKLYKMLTEIYTEDNFVKFFKVLNRKTYLNFDKAVFKINIVPKVNYTIYDGFNLRNTNLAANFNGQNTEINNMNFTKLKNFTGLFEFYKLLCVRGIITSKTKSLDKGYNKALNDLCIKVNNWDLFFSPSEDNFTNDLNKGEEITSDTNIEAAEENISLDLIQQYYLTFNFDNEPENISIENLSSDIIGQLELMPNIERFPNGKKYELDKYTMFHYLRAQEFEHGKSRIALTNSVNEALLNPSRVYTFFSSDYVKKVNKATEAAMFLGWVEQLVYDFTDETSEVSTTDKIADITIIIPYIGPALNIGNMLYKDDFVGALIFSGAVILLEFIPEIAIPVLGTFALVSYIANKVLTVQTIDNALSKRNEKWDEVYKYIVTNWLAKVNTQIDLIRKKMKEALENQAEATKAIINYQYNQYTEEEKNNINFNIDDLSSKLNESINKAMININKFLNQCSVSYLMNSMIPYGVKRLEDFDASLKDALLKYIYDNRGTLIGQVDRLKDKVNNTLSTDIPFQLSKYVDNQRLLSTFTEYIKNILNNIILNLRYKDNNLIDLSGYGAKVEVYDGVELNDKNQFKLTSSANSKIRVTQNQNIIFNSVFLDFSVSFWIRIPKYKNDGIQNYIHNEYTIINCMKNNSGWKISIRGNRIIWTLIDINGKTKSVFFEYNIREDISEYINRWFFVTITNNLNNAKIYINGKLESNTDIKDIREVIANGEIIFKLDGDIDRTQFIWMKYFSIFNTELSQSNIEERYKIQSYSEYLKDFWGNPLMYNKEYYMFNAGNKNSYIKLKKDSPVGEILTRSKYNQNSKYINYRDLYIGEKFIIRRKSNSQSINDDIVRKEDYIYLDFFNLNQEWRVYTYKYFKKEEMKLFLAPIYDSDEFYNTIQIKEYDEQPTYSCQLLFKKDEESTDEIGLIGIHRFYESGIVFEEYKDYFCISKWYLKEVKRKPYNLKLGCNWQFIPKDEGWTE

SEQ ID NO: 65 - protein, 1296 aa, Artificial Sequence
  Polypeptide Sequence of mrBoNT/A(0)
MPFVNKQFNYKDPVNGVDIAYIKIPNAGQMQPVKAFKIHNKIWVIPERDTFTNPEEGDLNPPPEAKQVPVSYYDSTYLSTDNEKDNYLKGVTKLFERIYSTDLGRMLLTSIVRGIPFWGGSTIDTELKVIDTNCINVIQPDGSYRSEELNLVIIGPSADIIQFECKSFGHEVLNLTRNGYGSTQYIRFSPDFTFGFEESLEVDTNPLLGAGKFATDPAVTLAHQLIYAGHRLYGIAINPNRVFKVNTNAYYEMSGLEVSFEELRTFGGHDAKFIDSLQENEFRLYYYNKFKDIASTLNKAKSIVGTTASLQYMKNVFKEKYLLSEDTSGKFSVDKLKFDKLYKMLTEIYTEDNFVKFFKVLNRKTYLNFDKAVFKINIVPKVNYTIYDGFNLRNTNLAANFNGQNTEINNMNFTKLKNFTGLFEFYKLLCVRGIITSKTKSLDKGYNKALNDLCIKVNNWDLFFSPSEDNFTNDLNKGEEITSDTNIEAAEENISLDLIQQYYLTFNFDNEPENISIENLSSDIIGQLELMPNIERFPNGKKYELDKYTMFHYLRAQEFEHGKSRIALTNSVNEALLNPSRVYTFFSSDYVKKVNKATEAAMFLGWVEQLVYDFTDETSEVSTTDKIADITIIIPYIGPALNIGNMLYKDDFVGALIFSGAVILLEFIPEIAIPVLGTFALVSYIANKVLTVQTIDNALSKRNEKWDEVYKYIVTNWLAKVNTQIDLIRKKMKEALENQAEATKAIINYQYNQYTEEEKNNINFNIDDLSSKLNESINKAMININKFLNQCSVSYLMNSMIPYGVKRLEDFDASLKDALLKYIYDNRGTLIGQVDRLKDKVNNTLSTDIPFQLSKYVDNQRLLSTFTEYIKNIINTSILNLRYESKHLIDLSRYASKINIGSKVNFDPIDKNQIQLFNLESSKIEVILKKAIVYNSMYENFSTSFWIRIPKYFNKISLNNEYTIINCMENNSGWKVSLNYGEIIWTLQDTKEIKQRVVFKYSQMINISDYINRWIFVTITNNRLNKSKIYINGRLIDQKPISNLGNIHASNKIMFKLDGCRDTHRYIWIKYFNLFDKELNEKEIKDLYDNQSNSGILKDFWGDYLQYDKPYYMLNLYDPNKYVDVNNVGIRGYMYLKGPRGSVMTTNIYLNSSLYRGTKFIIKKYASGNKDNIVRNNDRVYINVVVKNKEYRLATNASQAGVEKILSALEIPDVGNLSQVVVMKSKNDKGITNKCKMNLQDNNGNDIGFIGFHQFNNIAKLVASNWYNRQIERSSRTLGCSWEFIPVDDGWGERPL

SEQ ID NO: 66 - protein, 7 aa, Artificial Sequence
  Leucine-Based Motif
  SITE (1)..(1): Xaa can be any naturally occurring amino acid
  SITE (3)..(5): Xaa can be any naturally occurring amino acid
XDXXXLL

SEQ ID NO: 67 - protein, 7 aa, Artificial Sequence
  Leucine-Based Motif
  SITE (1)..(1): Xaa can be any naturally occurring amino acid
  SITE (3)..(5): Xaa can be any naturally occurring amino acid
XEXXXLL

SEQ ID NO: 68 - protein, 7 aa, Artificial Sequence
  Leucine-Based Motif
  SITE (1)..(1): Xaa can be any naturally occurring amino acid
  SITE (3)..(5): Xaa can be any naturally occurring amino acid
XEXXXIL

SEQ ID NO: 69 - protein, 7 aa, Artificial Sequence
  Leucine-Based Motif
  SITE (1)..(1): Xaa can be any naturally occurring amino acid
  SITE (3)..(5): Xaa can be any naturally occurring amino acid
XEXXXLM

SEQ ID NO: 70 - protein, 4 aa, Artificial Sequence
  Tyrosine-Based Motif
  SITE (2)..(3): Xaa can be any naturally occurring amino acid
  VARIANT (4)..(4): Xaa is a hydrophobic amino acid
YXXX

SEQ ID NO: 71 - protein, 6 aa, Clostridium botulinum
NIINTS

SEQ ID NO: 72 - protein, 6 aa, Clostridium botulinum
NIVNTS

SEQ ID NO: 73 - protein, 6 aa, Clostridium botulinum
NITNAS

SEQ ID NO: 74 - protein, 6 aa, Clostridium botulinum
NITNTS

SEQ ID NO: 75 - protein, 6 aa, Clostridium botulinum
EILNNI

SEQ ID NO: 76 - protein, 6 aa, Clostridium botulinum
DILNNI